European Patent Specification EP 3 310 911 B1, published March 15, 2023. Title: B. GIBSONII-CLADE SERINE PROTEASES. Applicant: Danisco US Inc. The sequence listing filed with the application follows.

SEQUENCE LISTING (257 sequences)

SEQ ID NO: 1 - DNA, 608 bp, B. subtilis
gaattctccattttcttctgctatcaaaataacagactcgtgattttccaaacgagctttcaaaaaagcctctgccccttgcaaatcggatgcctgtctataaaattcccgatattggttaaacagcggcgcaatggcggccgcatctgatgtctttgcttggcgaatgttcatcttatttcttcctccctctcaataattttttcattctatcccttttctgtaaagtttatttttcagaatacttttatcatcatgctttgaaaaaatatcacgataatatccattgttctcacggaagcacacgcaggtcatttgaacgaattttttcgacaggaatttgccgggactcaggagcatttaacctaaaaaagcatgacatttcagcataatgaacatttactcatgtctattttcgttcttttctgtatgaaaatagttatttcgagtctctacggaaatagcgagagatgatatacctaaatagagataaaatcatctcaaaaaaatgggtctactaaaatattattccatctattacaataaattcacagaatagtcttttaagtaagtctactctgaatttttttaaaaggagagggtaaaga

SEQ ID NO: 2 - DNA, 87 bp, B. subtilis
gtgagaagcaaaaaattgtggatcagcttgttgtttgcgttaacgttaatctttacgatggcgttcagcaacatgtctgctagcgca

SEQ ID NO: 3 - protein, 29 aa, B. subtilis
MRSKKLWISLLFALTLIFTMAFSNMSASA

SEQ ID NO: 4 - DNA, 261 bp, B. gibsonii
gcagaagaaaaagtaaaatacttaataggtttcgaagaagaagcagaacttgaagccttcactgaggaaattgaccaagttggtgtattttctgttgaagaacaaagtgtagctgaggatacgttagatattgatgtagacattattgatgaatatgattatattgatgtgttagctgtagaattagatcctgaggatgtagatgcgttaagtgaagaagcaggtatctcatttattgaagaagacattgaactgtctatt

SEQ ID NO: 5 - DNA, 252 bp, B. lentus
gctgaagaagcaaaagaaaaatatttaattggctttaatgagcaggaagctgtcagtgagtttgtagaacaagtagaggcaaatgacgaggtcgccattctctctgaggaagaggaagtcgaaattgaattgcttcatgaatttgaaacgattcctgttttatccgttgagttaagcccagaagatgtggacgcgcttgagctcgatccagcgatttcttatattgaagaggatgcagaagtaacgacaatg

SEQ ID NO: 6 - DNA, 807 bp, B. gibsonii
caacaaacagtgccatggggaattactcgtgtgcaagccccagctgttcataaccgtggaattacaggttctggtgtaagagttgctatcctcgattcaggtatttccacacatgaagacttaaatgttcgtggtggcgttagctttgtaccaggggaaccaacgactgctgatttaaatgggcatggcacgcatgtggctgggacggtagctgctttaaacaattcgattggcgttgttggcgtagcaccgtcagcggatctatacgctgttaaagtattaggggcgaatggtagaggttcggtcagcgggattgcccaaggattggaatgggcagcagcaaataacatgcacattgctaatatgagtttaggaagcgatgcaccaagttctacacttgagcgtgctgttaattatgcgacttctagagatgttcttgttattgcggcaactgggaataacggttctggctcagtaggctatccggcccgttatgcgaacgcaatggcagtcggagctactgaccaaaacaacagacgcgccaacttttcacagtatggcacggggattgacattgtcgcaccaggtgtaaacgtgcagagcacatacccaggtaaccgttatgtgagcatgaacggtacatcgatggctactcctcatgttgcaggtgcagcagcccttgttaaacaacgctatccatcttggaatgcgactcaaatccgcaatcatctaaagaatacggcaacgaatttaggaaactcttcacaatttggaagcggacttgtcaatgcagaagcggcaacacgc

SEQ ID NO: 7 - DNA, 42 bp, artificial sequence
  primer
gaggatgcagaagtaacgacaatgcaacaaacagtgccatgg

SEQ ID NO: 8 - DNA, 52 bp, artificial sequence
  primer
ccaaggccggttttttatgtatctagattagcgtgttgccgcttctgcattg

SEQ ID NO: 9 - DNA, 42 bp, artificial sequence
  primer
gaagaagacattgaactgtctattcaacaaacagtgccatgg

SEQ ID NO: 10 - DNA, 52 bp, artificial sequence
  primer
caatgcagaagcggcaacacgctaatctagatacataaaaaaccggccttgg

SEQ ID NO: 11 - DNA, 42 bp, artificial sequence
  primer
ccatggcactgtttgttgcattgtcgttacttctgcatcctc

SEQ ID NO: 12 - DNA, 42 bp, artificial sequence
  primer
ccatggcactgtttgttgaatagacagttcaatgtcttcttc

SEQ ID NO: 13 - DNA, 93 bp, artificial sequence
  terminator
ggttaccttgaatgtatataaacattctcaaagggatttctaataaaaaacgctcggttgccgccgggcgttttttatgcatcgatggaattc

SEQ ID NO: 14 - DNA, 21 bp, artificial sequence
  B. gibsonii-clade subtilisin
ggatcctgactgcctgagctt

SEQ ID NO: 15 - DNA, 1155 bp, artificial sequence
  B. gibsonii-clade subtilisin
atgagaagcaaaaaattgtggatcagcttgttgtttgcgttaacgttaatctttacgatggcgttcagcaacatgtctgctagcgcagcagaagaaaaagtaaaatacttaataggtttcgaagaagaagcagaacttgaagccttcactgaggaaattgaccaagttggtgtattttctgttgaagaacaaagtgtagctgaggatacgttagatattgatgtagacattattgatgaatatgattatattgatgtgttagctgtagaattagatcctgaggatgtagatgcgttaagtgaagaagcaggtatctcatttattgaagaagacattgaactgtctattcaacaaacagtgccatggggaattactcgtgtgcaagccccagctgttcataaccgtggaattacaggttctggtgtaagagttgctatcctcgattcaggtatttccacacatgaagacttaaatgttcgtggtggcgttagctttgtaccaggggaaccaacgactgctgatttaaatgggcatggcacgcatgtggctgggacggtagctgctttaaacaattcgattggcgttgttggcgtagcaccgtcagcggatctatacgctgttaaagtattaggggcgaatggtagaggttcggtcagcgggattgcccaaggattggaatgggcagcagcaaataacatgcacattgctaatatgagtttaggaagcgatgcaccaagttctacacttgagcgtgctgttaattatgcgacttctagagatgttcttgttattgcggcaactgggaataacggttctggctcagtaggctatccggcccgttatgcgaacgcaatggcagtcggagctactgaccaaaacaacagacgcgccaacttttcacagtatggcacggggattgacattgtcgcaccaggtgtaaacgtgcagagcacatacccaggtaaccgttatgtgagcatgaacggtacatcgatggctactcctcatgttgcaggtgcagcagcccttgttaaacaacgctatccatcttggaatgcgactcaaatccgcaatcatctaaagaatacggcaacgaatttaggaaactcttcacaatttggaagcggacttgtcaatgcagaagcggcaacacgc

SEQ ID NO: 16 - protein, 385 aa, artificial sequence
  B. gibsonii-clade subtilisin
MRSKKLWISLLFALTLIFTMAFSNMSASAAEEKVKYLIGFEEEAELEAFTEEIDQVGVFSVEEQSVAEDTLDIDVDIIDEYDYIDVLAVELDPEDVDALSEEAGISFIEEDIELSIQQTVPWGITRVQAPAVHNRGITGSGVRVAILDSGISTHEDLNVRGGVSFVPGEPTTADLNGHGTHVAGTVAALNNSIGVVGVAPSADLYAVKVLGANGRGSVSGIAQGLEWAAANNMHIANMSLGSDAPSSTLERAVNYATSRDVLVIAATGNNGSGSVGYPARYANAMAVGATDQNNRRANFSQYGTGIDIVAPGVNVQSTYPGNRYVSMNGTSMATPHVAGAAALVKQRYPSWNATQIRNHLKNTATNLGNSSQFGSGLVNAEAATR

SEQ ID NO: 17 - protein, 356 aa, artificial sequence
  B. gibsonii-clade subtilisin
AEEKVKYLIGFEEEAELEAFTEEIDQVGVFSVEEQSVAEDTLDIDVDIIDEYDYIDVLAVELDPEDVDALSEEAGISFIEEDIELSIQQTVPWGITRVQAPAVHNRGITGSGVRVAILDSGISTHEDLNVRGGVSFVPGEPTTADLNGHGTHVAGTVAALNNSIGVVGVAPSADLYAVKVLGANGRGSVSGIAQGLEWAAANNMHIANMSLGSDAPSSTLERAVNYATSRDVLVIAATGNNGSGSVGYPARYANAMAVGATDQNNRRANFSQYGTGIDIVAPGVNVQSTYPGNRYVSMNGTSMATPHVAGAAALVKQRYPSWNATQIRNHLKNTATNLGNSSQFGSGLVNAEAATR

SEQ ID NO: 18 - protein, 269 aa, artificial sequence
  B. gibsonii-clade subtilisin
QQTVPWGITRVQAPAVHNRGITGSGVRVAILDSGISTHEDLNVRGGVSFVPGEPTTADLNGHGTHVAGTVAALNNSIGVVGVAPSADLYAVKVLGANGRGSVSGIAQGLEWAAANNMHIANMSLGSDAPSSTLERAVNYATSRDVLVIAATGNNGSGSVGYPARYANAMAVGATDQNNRRANFSQYGTGIDIVAPGVNVQSTYPGNRYVSMNGTSMATPHVAGAAALVKQRYPSWNATQIRNHLKNTATNLGNSSQFGSGLVNAEAATR

SEQ ID NO: 19 - protein, 268 aa, B. gibsonii
QTVPWGITRVQAPAVHNRGITGSGVRVAILDSGISAHSDLNIRGGASFVPGEPTTADLNGHGTHVAGTVAALNNSIGVIGVAPNAELYAVKVLGANGSGSVSGIAQGLEWAATNNMHIANMSLGSDFPSSTLERAVNYATSRDVLVIAATGNNGSGSVGYPARYANAMAVGATDQNNRRANFSQYGTGIDIVAPGVNVQSTYPGNRYVSMNGTSMATPHVAGAAALVKQRYPSWNATQIRNHLKNTATNLGNSSQFGSGLVNAEAATR

SEQ ID NO: 20 - protein, 268 aa, artificial sequence
  B. gibsonii-clade subtilisin
QTVPWGITRVQAPAVHNRGITGSGVRVAILDSGISTHEDLNVRGGVSFVPGEPTTADLNGHGTHVAGTVAALNNSIGVVGVAPSADLYAVKVLGANGRGSVSGIAQGLEWAAANNMHIANMSLGSDAPSSTLERAVNYATSRDVLVIAATGNNGSGSVGYPARYANAMAVGATDQNNRRANFSQYGTGIDIVAPGVNVQSTYPGNRYVSMNGTSMATPHVAGAAALVKQRYPSWNATQIRNHLKNTATNLGNSSQFGSGLVNAEAATR

SEQ ID NO: 21 - DNA, 807 bp, artificial sequence
  B. gibsonii-clade subtilisin
caacaaacagtgccatggggaattactcgtgtgcaagccccagctgttcataaccgtggaattacaggttctggtgtaagagttgctatcctcgattcaggtatttccacacatgaagacttaaatattcgtggtggcgttagctttgtaccaggggaaccaacgactgctgatttaaatgggcatggcacgcatgtggctgggacggtagctgctttagacaattcgattggcgttgttggcgtagcaccgtcagcggatctatacgctgttaaagtattaggggcgaatggtagaggttcgattagcgggattgcccaaggattggaatgggcagcacaaaataacatgcacattgctaatatgagtttaggaacagatgcaccaagttctacacttgagcgtgctgttaattatgcgacttctagagatgttcttgttattgcggcaactgggaataacggttctggcacagtaggctatccggcccgttatgcgaacgcaatggcagtcggagctactgaccaaaacaacagacgcgccaacttttcacagtatggcacggggattgacattgtcgcaccaggtgtaaacgtgcagagcacatacccaggtaaccgttatgtgagcatgaacggtacatcgatggctactcctcatgttgcaggtgcagcagcccttgttaaacaacgctatccatcttggaatgcgactcaaatccgcgaccatctaaagaatacggcaacgaatttaggaaactcttcacaatttggaagcggacttgtcaatgcagaagcggcaacacgc

SEQ ID NO: 22 - protein, 269 aa, artificial sequence
  B. gibsonii-clade subtilisin
QQTVPWGITRVQAPAVHNRGITGSGVRVAILDSGISTHEDLNIRGGVSFVPGEPTTADLNGHGTHVAGTVAALDNSIGVVGVAPSADLYAVKVLGANGRGSISGIAQGLEWAAQNNMHIANMSLGTDAPSSTLERAVNYATSRDVLVIAATGNNGSGTVGYPARYANAMAVGATDQNNRRANFSQYGTGIDIVAPGVNVQSTYPGNRYVSMNGTSMATPHVAGAAALVKQRYPSWNATQIRDHLKNTATNLGNSSQFGSGLVNAEAATR

SEQ ID NO: 23 - DNA, 807 bp, artificial sequence
  B. gibsonii-clade subtilisin
caacaaacagtgccatggggaattactcgtgtgcaagccccagctgttcataaccgtggaattacaggttctggtgtaagagttgctatcctcgattcaggtatttccacacatgaagacttaaatgttcgtggtggcgttagctttgtaccaggggaaccaggcactgctgatttaaatgggcatggcacgcatgtggctgggacggtagctgctttagacaattcgattggcgttgttggcgtagcaccgaacgcggaactatacgctgttaaagtattaggggcgaatggtagaggttcgattagcgggattgcccaaggattggaatgggcagcacaaaataacatgcacattgctaatatgagtttaggaacagatgcaccaagttctacacttgagcgtgctgttaattatgcgacttctagagatgttcttgttattgcggcaactgggaataacggttctggctcagtaggctatccggcccgttatgcgaacgcaatggcagtcggagctactgaccaaaacaacagacgcgccaacttttcacagtatggcacggggattgacattgtcgcaccaggtgtaaacgtgcagagcacatacccaggtaaccgttatgtgagcatgaacggtacatcgatggctactcctcatgttgcaggtgcagcagcccttgttaaacaacgctatccatcttggaatgcgactcaaatccgcaatcatctaaagaatacggcaacgaatttaggaaactcttcacaatttggaagcggacttgtcaatgcagaagcggcaacacgc

SEQ ID NO: 24 - protein, 269 aa, artificial sequence
  B. gibsonii-clade subtilisin
QQTVPWGITRVQAPAVHNRGITGSGVRVAILDSGISTHEDLNVRGGVSFVPGEPGTADLNGHGTHVAGTVAALDNSIGVVGVAPNAELYAVKVLGANGRGSISGIAQGLEWAAQNNMHIANMSLGTDAPSSTLERAVNYATSRDVLVIAATGNNGSGSVGYPARYANAMAVGATDQNNRRANFSQYGTGIDIVAPGVNVQSTYPGNRYVSMNGTSMATPHVAGAAALVKQRYPSWNATQIRNHLKNTATNLGNSSQFGSGLVNAEAATR

SEQ ID NO: 25 - DNA, 807 bp, artificial sequence
  B. gibsonii-clade subtilisin
caacaaacagtgccatggggaattactcgtgtgcaagccccagctgttcataaccgtggaattacaggttctggtgtaagagttgctatcctcgattcaggtatttccacacatgaagacttaacaattcgtggtggcgctagctttgtaccaggggaaccaacgactgctgatttaaatgggcatggcacgcatgtggctgggacggtagctgctttagacaattcgattggcgttattggcgtagcaccgaacgcggaactatacgctgttaaagtattaggggcgaatggtagaggttcgattagcgggattgcccaaggattggaatgggcagcaaccaataacatgcacattgctaatatgagtttaggaacagatgcaccaagttctacacttgagcgtgctgttaattatgcgacttctagagatgttcttgttattgcggcaactgggaataacggttctggcacagtaggctatccggcccgttatgcgaacgcaatggcagtcggagctactgaccaaaacaacagacgcgccaacttttcacagtatggcacggggattgacattgtcgcaccaggtgtaaacgtgcagagcacatacccaggtaaccgttatgtgagcatgaacggtacatcgatggctactcctcatgttgcaggtgcagcagcccttgttaaacaacgctatccatcttggaatgcgactcaaatccgcgaccatctaaagaatacggcaacgaatttaggaaactcttcacaatttggaagcggacttgtcaatgcagaagcggcaacacgc

SEQ ID NO: 26 - protein, 269 aa, artificial sequence
  B. gibsonii-clade subtilisin
QQTVPWGITRVQAPAVHNRGITGSGVRVAILDSGISTHEDLTIRGGASFVPGEPTTADLNGHGTHVAGTVAALDNSIGVIGVAPNAELYAVKVLGANGRGSISGIAQGLEWAATNNMHIANMSLGTDAPSSTLERAVNYATSRDVLVIAATGNNGSGTVGYPARYANAMAVGATDQNNRRANFSQYGTGIDIVAPGVNVQSTYPGNRYVSMNGTSMATPHVAGAAALVKQRYPSWNATQIRDHLKNTATNLGNSSQFGSGLVNAEAATR

SEQ ID NO: 27 - DNA, 807 bp, artificial sequence
  B. gibsonii-clade subtilisin
caacaaacagtgccatggggaattactcgtgtgcaagccccagctgttcataaccgtggaattacaggttctggtgtaagagttgctatcctcgattcaggtatttccacacatgaagacttaaatgttcgtggtggcgttagctttgtaccaggggaaccaacgactgctgatttaaatgggcatggcacgcatgtggctgggacggtagctgctttagacaattcgattggcgttgttggcgtagcaccgaacgcggaactatacgctgttaaagtattaggggcgaatggtagaggttcgattagcgggattgcccaaggattggaatgggcagcacaaaataacatgcacattgctaatatgagtttaggaacagatgcaccaagttctacacttgagcgtgctgttaattatgcgacttctagagatgttcttgttattgcggcaactgggaataacggttctggctcagtaggctatccggcccgttatgcgaacgcaatggcagtcggagctactgaccaaaacaacagacgcgccaacttttcacagtatggcacggggattgacattgtcgcaccaggtgtaaacgtgcagagcacatacccaggtaaccgttatgtgagcatgaacggtacatcgatggctactcctcatgttgcaggtgcagcagcccttgttaaacaacgctatccatcttggaatgcgactcaaatccgcgaccatctaaagaatacggcaacgaatttaggaaactcttcacaatttggaagcggacttgtcaatgcagaagcggcaacacgc

SEQ ID NO: 28 - protein, 269 aa, artificial sequence
  B. gibsonii-clade subtilisin
QQTVPWGITRVQAPAVHNRGITGSGVRVAILDSGISTHEDLNVRGGVSFVPGEPTTADLNGHGTHVAGTVAALDNSIGVVGVAPNAELYAVKVLGANGRGSISGIAQGLEWAAQNNMHIANMSLGTDAPSSTLERAVNYATSRDVLVIAATGNNGSGSVGYPARYANAMAVGATDQNNRRANFSQYGTGIDIVAPGVNVQSTYPGNRYVSMNGTSMATPHVAGAAALVKQRYPSWNATQIRDHLKNTATNLGNSSQFGSGLVNAEAATR

SEQ ID NO: 29 - DNA, 807 bp, artificial sequence
  B. gibsonii-clade subtilisin
caacaaacagtgccatggggaattactcgtgtgcaagccccagctgttcataaccgtggaattacaggttctggtgtaaaagttgctatcctcgattcaggtatttccacacatgaagacttaaatattcgtggtggcgttagctttgtaccaggggaaccaggctatgctgatttaaatgggcatggcacgcatgtggctgggacggtagctgctttagacaattcgattggcgttattggcgtagcaccgaacgcggaactatacgctgttaaagtattaggggcgaatggtagaggttcgattagcgggattgcccaaggattggaatgggcagcaaccaataacatgcacattgctaatatgagtttaggaacagatgcaccaagttctacacttgagcgtgctgttaattatgcgacttctagagatgttcttgttattgcggcaactgggaataacggttctggctcagtaggctatccggcccgttatgcgaacgcaatggcagtcggagctactgaccaaaacaacagacgcgccaacttttcacagtatggcacggggattgacattgtcgcaccaggtgtaaacgtgcagagcacatacccaggtaaccgttatgtgagcatgaacggtacatcgatggctactcctcatgttgcaggtgcagcagcccttgttaaacaacgctatccatcttggaatgcgactcaaatccgcgaccatctaaagaatacggcaacgaatttaggaaactcttcacaatttggaagcggacttgtcaatgcagaagcggcaacacgc

SEQ ID NO: 30 - protein, 269 aa, artificial sequence
  B. gibsonii-clade subtilisin
QQTVPWGITRVQAPAVHNRGITGSGVKVAILDSGISTHEDLNIRGGVSFVPGEPGYADLNGHGTHVAGTVAALDNSIGVIGVAPNAELYAVKVLGANGRGSISGIAQGLEWAATNNMHIANMSLGTDAPSSTLERAVNYATSRDVLVIAATGNNGSGSVGYPARYANAMAVGATDQNNRRANFSQYGTGIDIVAPGVNVQSTYPGNRYVSMNGTSMATPHVAGAAALVKQRYPSWNATQIRDHLKNTATNLGNSSQFGSGLVNAEAATR

SEQ ID NO: 31 - DNA, 807 bp, artificial sequence
  B. gibsonii-clade subtilisin
caacaaacagtgccatggggaattactcgtgtgcaagccccagctgttcataaccgtggaattacaggttctggtgtaagagttgctatcctcgactcaggtatttccacacatgaagacttaacaattcgtggtggcgttagctttgtaccaggggaaccaacgtatgctgatttaaatgggcatggcacgcatgtggctgggacggtagctgctttagacaattcgattggcgttgttggcgtagcaccgtcagcggatctatacgctgttaaagtattaggggcgaatggtagaggttcggtcagcgggattgcccaaggattggaatgggcagcacaaaataacatgcacattgctaatatgagtttaggaacagatgcaccaagttctacacttgagcgtgctgttaattatgcgacttctagagatgttcttgttattgcggcaactgggaataacggttctggctcagtaggctatccggcccgttatgcgaacgcaatggcagtcggagctactgaccaaaacaacagacgcgccaacttttcacagtatggcacggggattgacattgtcgcaccaggtgtaaacgtgcagagcacatacccaggtaaccgttatgtgagcatgaacggtacatcgatggctactcctcatgttgcaggtgcagcagcccttgttaaacaacgctatccatcttggaatgcgactcaaatccgcaatcatctaaagaatacggcaacgaatttaggaaactcttcacaatttggaagcggacttgtcaatgcagaagcggcaacacgc

SEQ ID NO: 32 - protein, 269 aa, artificial sequence
  B. gibsonii-clade subtilisin
QQTVPWGITRVQAPAVHNRGITGSGVRVAILDSGISTHEDLTIRGGVSFVPGEPTYADLNGHGTHVAGTVAALDNSIGVVGVAPSADLYAVKVLGANGRGSVSGIAQGLEWAAQNNMHIANMSLGTDAPSSTLERAVNYATSRDVLVIAATGNNGSGSVGYPARYANAMAVGATDQNNRRANFSQYGTGIDIVAPGVNVQSTYPGNRYVSMNGTSMATPHVAGAAALVKQRYPSWNATQIRNHLKNTATNLGNSSQFGSGLVNAEAATR

SEQ ID NO: 33 - DNA, 807 bp, artificial sequence
  B. gibsonii-clade subtilisin
caacaaacagtgccatggggaattactcgtgtgcaagccccagctgttcataaccgtggaattacaggttctggtgtaagagttgctatcctcgattcaggtatttccacacatgaagacttaaatgttcgtggtggcgttagctttgtaccaggggaaccaggctatgctgatttaaatgggcatggcacgcatgtggctgggacggtagctgctttagacaattcgattggcgttgttggcgtagcaccgtcagcggatctatacgctgttaaagtattaggggcgaatggtagaggttcgattagcgggattgcccaaggattggaatgggcagcacaaaataacatgcacattgctaatatgagtttaggaacagatgcaccaagttctacacttgagcgtgctgttaattatgcgacttctagagatgttcttgttattgcggcaactgggaataacggttctggctcagtaggctatccggcccgttatgcgaacgcaatggcagtcggagctactgaccaaaacaacagacgcgccaacttttcacagtatggcacggggattgacattgtcgcaccaggtgtaaacgtgcagagcacatacccaggtaaccgttatgtgagcatgaacggtacatcgatggctactcctcatgttgcaggtgcagcagcccttgttaaacaacgctatccatcttggaatgcgactcaaatccgcgaccatctaaagaatacggcaacgaatttaggaaactcttcacaatttggaagcggacttgtcaatgcagaagcggcaacacgc

SEQ ID NO: 34 - protein, 269 aa, artificial sequence
  B. gibsonii-clade subtilisin
QQTVPWGITRVQAPAVHNRGITGSGVRVAILDSGISTHEDLNVRGGVSFVPGEPGYADLNGHGTHVAGTVAALDNSIGVVGVAPSADLYAVKVLGANGRGSISGIAQGLEWAAQNNMHIANMSLGTDAPSSTLERAVNYATSRDVLVIAATGNNGSGSVGYPARYANAMAVGATDQNNRRANFSQYGTGIDIVAPGVNVQSTYPGNRYVSMNGTSMATPHVAGAAALVKQRYPSWNATQIRDHLKNTATNLGNSSQFGSGLVNAEAATR

SEQ ID NO: 35 - DNA, 807 bp, artificial sequence
  B. gibsonii-clade subtilisin
caacaaacagtgccatggggaattactcgtgtgcaagccccagctgttcataaccgtggaattacaggttctggtgtaagagttgctatcctcgattcaggtatttccacacatgaagacttaaatgttcgtggtggcgttagctttgtaccaggggaaccaggcactgctgatttaaatgggcatggcacgcatgtggctgggacggtagctgctttaaacaattcgattggcgttgttggcgtagcaccgtcagcggatctatacgctgttaaagtattaggggcgaatggtagaggttcgattagcgggattgcccaaggattggaatgggcagcagcaaataacatgcacattgctaatatgagtttaggaacagatgcaccaagttctacacttgagcgtgctgttaattatgcgacttctagagatgttcttgttattgcggcaactgggaataacggttctggcacagtaggctatccggcccgttatgcgaacgcaatggcagtcggagctactgaccaaaacaacagacgcgccaacttttcacagtatggcacggggattgacattgtcgcaccaggtgtaaacgtgcagagcacatacccaggtaaccgttatgtgagcatgaacggtacatcgatggctactcctcatgttgcaggtgcagcagcccttgttaaacaacgctatccatcttggaatgcgactcaaatccgcaatcatctaaagaatacggcaacgaatttaggaaactcttcacaatttggaagcggacttgtcaatgcagaagcggcaacacgc

SEQ ID NO: 36 - protein, 269 aa, artificial sequence
  B. gibsonii-clade subtilisin
QQTVPWGITRVQAPAVHNRGITGSGVRVAILDSGISTHEDLNVRGGVSFVPGEPGTADLNGHGTHVAGTVAALNNSIGVVGVAPSADLYAVKVLGANGRGSISGIAQGLEWAAANNMHIANMSLGTDAPSSTLERAVNYATSRDVLVIAATGNNGSGTVGYPARYANAMAVGATDQNNRRANFSQYGTGIDIVAPGVNVQSTYPGNRYVSMNGTSMATPHVAGAAALVKQRYPSWNATQIRNHLKNTATNLGNSSQFGSGLVNAEAATR

SEQ ID NO: 37 - DNA, 807 bp, artificial sequence
  B. gibsonii-clade subtilisin
caacaaacagtgccatggggaattactcgtgtgcaagccccagctgttcataaccgtggaattacaggttctggtgtaagagttgctatcctcgattcaggtatttccacacatgaagacttaaatgttcgtggtggcgttagctttgtaccaggggaaccaacgactgctgatttaaatgggcatggcacgcatgtggctgggacggtagctgctttaaacaattcgattggcgttgttggcgtagcaccgtcagcggatctatacgctgttaaagtattaggggcgaatggtagaggttcggtcagcgggattgcccaaggattggaatgggcagcagcaaataacatgcacattgctaatatgagtttaggaacagatgcaccaagttctacacttgagcgtgctgttaattatgcgacttctagagatgttcttgttattgcggcaactgggaataacggttctggctcagtaggctatccggctcgttatgcgaacgcaatggcagtcggagctactgaccaaaacaacagacgcgccaacttttcacagtatggcacggggattgacattgtcgcaccaggtgtaaacgtgcagagcacatacccaggtaaccgttatgtgagcatgaacggtacatcgatggctactcctcatgttgcaggtgcagcagcccttgttaaacaacgctatccatcttggaatgcgactcaaatccgcgaccatctaaagaatacggcaacgaatttaggaaactcttcacaatttggaagcggacttgtcaatgcagaagcggcaacacgc

SEQ ID NO: 38 - protein, 269 aa, artificial sequence
  B. gibsonii-clade subtilisin
QQTVPWGITRVQAPAVHNRGITGSGVRVAILDSGISTHEDLNVRGGVSFVPGEPTTADLNGHGTHVAGTVAALNNSIGVVGVAPSADLYAVKVLGANGRGSVSGIAQGLEWAAANNMHIANMSLGTDAPSSTLERAVNYATSRDVLVIAATGNNGSGSVGYPARYANAMAVGATDQNNRRANFSQYGTGIDIVAPGVNVQSTYPGNRYVSMNGTSMATPHVAGAAALVKQRYPSWNATQIRDHLKNTATNLGNSSQFGSGLVNAEAATR

SEQ ID NO: 39 - DNA, 807 bp, artificial sequence
  B. gibsonii-clade subtilisin
caacaaacagtgccatggggaattactcgtgtgcaagccccagctgttcataaccgtggaattacaggttctggtgtaagagttgctatcctcgattcaggtatttccacacatgaagacttaaatgttcgtggtggcgttagctttgtaccaggggaaccaacgactgctgatttaaatgggcatggcacgcatgtggctgggacggtagctgctttaaacaattcgattggcgttgttggcgtagcaccgtcagcggatctatacgctgttaaagtattaggggcgaatggtagaggttcggtcagcgggattgcccaaggattggaatgggcagcacaaaataacatgcacattgctaatatgagtttaggaacagatgcaccaagttctacacttgagcgtgctgttaattatgcgacttctgcagatgttcttgttattgcggcaactgggaataacggttctggctcagtaggctatccggcccgttatgcgaacgcaatggcagtcggagctactgaccaaaacaacagacgcgccaacttttcacagtatggcacggggattgacattgtcgcaccaggtgtaaacgtgcagagcacatacccaggtaaccgttatgtgagcatgaacggtacatcgatggctactcctcatgttgcaggtgcagcagcccttgttaaacaacgctatccatcttggaatgcgactcaaatccgcaatcatctaaagaatacggcaacgaatttaggaaactcttcacaatttggaagcggacttgtcaatgcagaagcggcaacacgc

SEQ ID NO: 40 - protein, 269 aa, artificial sequence
  B. gibsonii-clade subtilisin
QQTVPWGITRVQAPAVHNRGITGSGVRVAILDSGISTHEDLNVRGGVSFVPGEPTTADLNGHGTHVAGTVAALNNSIGVVGVAPSADLYAVKVLGANGRGSVSGIAQGLEWAAQNNMHIANMSLGTDAPSSTLERAVNYATSADVLVIAATGNNGSGSVGYPARYANAMAVGATDQNNRRANFSQYGTGIDIVAPGVNVQSTYPGNRYVSMNGTSMATPHVAGAAALVKQRYPSWNATQIRNHLKNTATNLGNSSQFGSGLVNAEAATR

SEQ ID NO: 41 - DNA, 807 bp, artificial sequence
  B. gibsonii-clade subtilisin
caacaaacagtgccatggggaattactcgtgtgcaagccccagctgttcataaccgtggaattacaggttctggtgtaagagttgctatcctcgattcaggtatttccacacatgaagacttaaatgttcgtggtggcgttagctttgtaccaggggaaccaacgactgctgatttaaatgggcatggcacgcatgtggctgggactgtagctgctttaaacaattcgattggcgttgttggcgtagcaccgtcagcggatctatacgctgttaaagtattaggggcgaatggtagaggttcggtcagcgggattgcccaaggattggaatgggcagcacaaaataacatgcacattgctaatatgagtttaggaagcgatgcaccaagttctacacttgagcgtgctgttaattatgcgacttctagagatgttcttgttattgcggcaactgggaataacggttctggctcagtaggctatccggcccgttatgcgaacgcaatggcagtcggagctactgaccaaaacaacagacgcgccaacttttcacagtatggcacggggattgacattgtcgcaccaggtgtaaacgtgcagagcacatacccaggtaaccgttatgtgagcatgaacggtacatcgatggctactcctcatgttgcaggtgcagcagcccttgttaaacaacgctatccatcttggaatgcgactcaaatccgcgaccatctaaagaatacggcaacgaatttaggaaactcttcacaatttggaagcggacttgtcaatgcagaagcggcaacacgc

SEQ ID NO: 42 - protein, 269 aa, artificial sequence
  B. gibsonii-clade subtilisin
QQTVPWGITRVQAPAVHNRGITGSGVRVAILDSGISTHEDLNVRGGVSFVPGEPTTADLNGHGTHVAGTVAALNNSIGVVGVAPSADLYAVKVLGANGRGSVSGIAQGLEWAAQNNMHIANMSLGSDAPSSTLERAVNYATSRDVLVIAATGNNGSGSVGYPARYANAMAVGATDQNNRRANFSQYGTGIDIVAPGVNVQSTYPGNRYVSMNGTSMATPHVAGAAALVKQRYPSWNATQIRDHLKNTATNLGNSSQFGSGLVNAEAATR

SEQ ID NO: 43 - DNA, 807 bp, artificial sequence
  B. gibsonii-clade subtilisin
caacaaacagtgccatggggaattactcgtgtgcaagccccagctgttcataaccgtggaattacaggttctggtgtaagagttgctatcctcgattcaggtatttccacacatgaagacttaaatgttcgtggtggcgttagctttgtaccaggggaaccaacgtatgctgatttaaatgggcatggcacgcatgtggctgggacggtagctgctttaaacaattcgattggcgttgttggcgtagcaccgtcagcggatctatacgctgttaaagtattaggggcgaatggtagaggttcggtcagcgggattgcccaaggattggaatgggcagcacaaaataacatgcacattgctaatatgagtttaggaacagatgcaccaagttctacacttgagcgtgctgttaattatgcgacttctagagatgttcttgttattgcggcaactgggaataacggttctggcacagtaggctatccggcccgttatgcgaacgcaatggcagtcggagctactgaccaaaacaacagacgcgccaacttttcacagtatggcacggggattgacattgtcgcaccaggtgtaaacgtgcagagcacatacccaggtaaccgttatgtgagcatgaacggtacatcgatggctactcctcatgttgcaggtgcagcagcccttgttaaacaacgctatccatcttggaatgcgactcaaatccgcgaccatctaaagaatacggcaacgaatttaggaaactcttcacaatttggaagcggacttgtcaatgcagaagcggcaacacgc

SEQ ID NO: 44 - protein, 269 aa, artificial sequence
  B. gibsonii-clade subtilisin
QQTVPWGITRVQAPAVHNRGITGSGVRVAILDSGISTHEDLNVRGGVSFVPGEPTYADLNGHGTHVAGTVAALNNSIGVVGVAPSADLYAVKVLGANGRGSVSGIAQGLEWAAQNNMHIANMSLGTDAPSSTLERAVNYATSRDVLVIAATGNNGSGTVGYPARYANAMAVGATDQNNRRANFSQYGTGIDIVAPGVNVQSTYPGNRYVSMNGTSMATPHVAGAAALVKQRYPSWNATQIRDHLKNTATNLGNSSQFGSGLVNAEAATR

SEQ ID NO: 45 - DNA, 807 bp, artificial sequence
  B. gibsonii-clade subtilisin
caacaaacagtgccatggggaattactcgtgtgcaagccccagctgttcataaccgtggaattacaggttctggtgtaagagttgctatcctcgattcaggtatttccacacatgaagacttaacagtttcaggtggcgttagctttgtaccaggggaaccaacgactgctgatttaaatgggcatggcacgcatgtggctgggacggtagctgctttagacaattcgattggcgttgttggcgtagcaccgtcagcggatctatacgctgttaaagtattaggggcgaatggtagaggttcggtcagcgggattgcccaaggattggaatgggcagcagcaaataacatgcacattgctaatatgagtttaggaacagatgcaccaagttctacacttgagcgtgctgttaattatgcgacttctagagatgttcttgttattgcggcaactgggaataacggttctggctcagtaggctatccggcccgttatgcgaacgcaatggcagtcggagctactgaccaaaacaacagacgcgccaacttttcacagtatggcacggggattgacattgtcgcaccaggtgtaaacgtgcagagcacatacccaggtaaccgttatgtgagcatgaacggtacatcgatggctactcctcatgttgcaggtgcagcagcccttgttaaacaacgctatccatcttggaatgcgactcaaatccgcaatcatctaaagaatacggcaacgaatttaggaaactcttcacaatttggaagcggacttgtcaatgcagaagcggcaacacgc

SEQ ID NO: 46 - protein, 269 aa, artificial sequence
  B. gibsonii-clade subtilisin
QQTVPWGITRVQAPAVHNRGITGSGVRVAILDSGISTHEDLTVSGGVSFVPGEPTTADLNGHGTHVAGTVAALDNSIGVVGVAPSADLYAVKVLGANGRGSVSGIAQGLEWAAANNMHIANMSLGTDAPSSTLERAVNYATSRDVLVIAATGNNGSGSVGYPARYANAMAVGATDQNNRRANFSQYGTGIDIVAPGVNVQSTYPGNRYVSMNGTSMATPHVAGAAALVKQRYPSWNATQIRNHLKNTATNLGNSSQFGSGLVNAEAATR

SEQ ID NO: 47-48 - skipped (2 entries)

SEQ ID NO: 49 - DNA, 807 bp, artificial sequence
  B. gibsonii-clade subtilisin
caacaaacagtgccatggggaattactcgtgtgcaagccccagctgttcataaccgtggaattacaggttctggtgtaagagttgctatcctcgattcaggtatttccacacatgaagacttaacagtttcaggtggcgttagctttgtaccaggggaaccaacgactgctgatttaaatgggcatggcacgcatgtggctgggacggtagctgctttaaacaattcgattggcgttgttggcgtagcaccgtcagcggatctatacgctgttaaagtattaggggcgaatggtagaggttcggtcagcgggattgcccaaggattggaatgggcagcagcaaataacatgcacattgctaatatgagtttaggaacagatgcaccaagttctacacttgagcgtgctgttaattatgcgacttctagagatgttcttgttattgcggcaactgggaataacggttctggctcagtaggctatccggcccgttatgcgaacgcaatggcagtcggagctactgaccaaaacaacagacgcgccaacttttcacagtatggcacggggattgacattgtcgcaccaggtgtaaacgtgcagagcacatacccaggtaaccgttatgtgagcatgaacggtacatcgatggctactcctcatgttgcaggtgcagcagcccttgttaaacaacgctatccatcttggaatgcgactcaaatccgcgaccatctaaagaatacggcaacgaatttaggaaactcttcacaatttggaagcggacttgtcaatgcagaagcggcaacacgc

SEQ ID NO: 50 - protein, 269 aa, artificial sequence
  B. gibsonii-clade subtilisin
QQTVPWGITRVQAPAVHNRGITGSGVRVAILDSGISTHEDLTVSGGVSFVPGEPTTADLNGHGTHVAGTVAALNNSIGVVGVAPSADLYAVKVLGANGRGSVSGIAQGLEWAAANNMHIANMSLGTDAPSSTLERAVNYATSRDVLVIAATGNNGSGSVGYPARYANAMAVGATDQNNRRANFSQYGTGIDIVAPGVNVQSTYPGNRYVSMNGTSMATPHVAGAAALVKQRYPSWNATQIRDHLKNTATNLGNSSQFGSGLVNAEAATR

SEQ ID NO: 51 - DNA, 807 bp, artificial sequence
  B. gibsonii-clade subtilisin
caacaaacagtgccatggggaattactcgtgtgcaagccccagctgttcataaccgtggaattacaggttctggtgtaagagttgctatcctcgattcaggtatttccacacatgaagacttaaatgttcgtggtggcgttagctttgtaccaggggaaccaggcactgctgatttaaatgggcatggcacgcatgtggctgggacggtagctgctttaaacaattcgattggcgttgttggcgtagcaccgtcagcggatctatacgctgttaaagtattaggggcgaatggtagaggttcggtcagcgggattgcccaaggattggaatgggcagcacaaaataacatgcacattgctaatatgagtttaggaacagatgcaccaagttctacacttgagcgtgctgttaattatgcgacttctagagatgttcttgttattgcggcaactgggaataacggttctggctcagtaggctatccggcccgttatgcgaacgcaatggcagtcggagctactgaccaaaacaacagacgcgccaacttttcacagtatggcacggggattgacattgtcgcaccaggtgtaaacgtgcagagcacatacccaggtaaccgttatgtgagcatgaacggtacatcgatggctactcctcatgttgcaggtgcagcagcccttgttaaacaacgctatccatcttggaatgcgactcaaatccgcaatcatctaaagaatacggcaacgaatttaggaaactcttcacaatttggaagcggacttgtcaatgcagaagcggcaacacgc

SEQ ID NO: 52 - protein, 269 aa, artificial sequence
  B. gibsonii-clade subtilisin
QQTVPWGITRVQAPAVHNRGITGSGVRVAILDSGISTHEDLNVRGGVSFVPGEPGTADLNGHGTHVAGTVAALNNSIGVVGVAPSADLYAVKVLGANGRGSVSGIAQGLEWAAQNNMHIANMSLGTDAPSSTLERAVNYATSRDVLVIAATGNNGSGSVGYPARYANAMAVGATDQNNRRANFSQYGTGIDIVAPGVNVQSTYPGNRYVSMNGTSMATPHVAGAAALVKQRYPSWNATQIRNHLKNTATNLGNSSQFGSGLVNAEAATR

SEQ ID NO: 53 - DNA, 807 bp, artificial sequence
  B. gibsonii-clade subtilisin
caacaaacagtgccatggggaattactcgtgtgcaagccccagctgttcataaccgtggaattacaggttctggtgtaaaagttgctatcctcgattcaggtatttccacacatgaagacttaaatgttcgtggtggcgttagctttgtaccaggggaaccaacgtatgctgatttaaatgggcatggcacgcatgtggctgggacggtagctgctttaaacaattcgattggcgttgttggcgtagcaccgtcagcggatctatacgctgttaaagtattaggggcgaatggtagaggttcggtcagcgggattgcccaaggattggaatgggcagcacaaaataacatgcacattgctaatatgagtttaggaacagatgcaccaagttctacacttgagcgtgctgttaattatgcgacttctagagatgttcttgttattgcggcaactgggaataacggttctggcacagtaagctatccggcccgttatgcgaacgcaatggcagtcggagctactgaccaaaacaacagacgcgccaacttttcacagtatggcacggggattgacattgtcgcaccaggtgtaaacgtgcagagcacatacccaggtaaccgttatgtgagcatgaacggtacatcgatggctactcctcatgttgcaggtgcagcagcccttgttaaacaacgctatccatcttggaatgcgactcaaatccgcgaccatctaaagaatacggcaacgaatttaggaaactcttcacaatatggaagcggacttgtcaatgcagaagcggcaacacgc

SEQ ID NO: 54 - protein, 269 aa, artificial sequence
  B. gibsonii-clade subtilisin
QQTVPWGITRVQAPAVHNRGITGSGVKVAILDSGISTHEDLNVRGGVSFVPGEPTYADLNGHGTHVAGTVAALNNSIGVVGVAPSADLYAVKVLGANGRGSVSGIAQGLEWAAQNNMHIANMSLGTDAPSSTLERAVNYATSRDVLVIAATGNNGSGTVSYPARYANAMAVGATDQNNRRANFSQYGTGIDIVAPGVNVQSTYPGNRYVSMNGTSMATPHVAGAAALVKQRYPSWNATQIRDHLKNTATNLGNSSQYGSGLVNAEAATR

SEQ ID NO: 55 - DNA, 807 bp, artificial sequence
  B. gibsonii-clade subtilisin
caacaaacagtgccatggggaattactcgtgtgcaagccccagctgttcataaccgtggaattacaggttctggtgtaagagttgctatcctcgattcaggtatttccacacatgaagacttaaatgttcgtggtggcgttagctttgtaccaggggaaccaacgactgctgatttaaatgggcatggcacgcatgtggctgggacggtagctgctttagacaattcgattggcgttgttggcgtagcaccgtcagcggatctatacgctgttaaagtattaggggcgaatggtagaggttcggtcagcgggattgcccaaggattggaatgggcagcagcaaataacatgcacattgctaatatgagtttaggaacagatgcaccaagttctacacttgagcgtgctgttaattatgcgacttctagagatgttcttgttattgcggcaactgggaataacggttctggctcagtaggctatccggcccgttatgcgaacgcaatggcagtcggagctactgaccaaaacaacagacgcgccaacttttcacagtatggcacggggattgacattgtcgcaccaggtgtaaacgtgcagagcacatacccaggtaaccgttatgtgagcatgaacggtacatcgatggctactcctcatgttgcaggtgcagcagcccttgttaaacaacgctatccatcttggaatgcgactcaaatccgcgaccatctaaagaatacggcaacgaatttaggaaactcttcacaatttggaagcggacttgtcaatgcagaagcggcaacacgc

SEQ ID NO: 56 - protein, 269 aa, artificial sequence
  B. gibsonii-clade subtilisin
QQTVPWGITRVQAPAVHNRGITGSGVRVAILDSGISTHEDLNVRGGVSFVPGEPTTADLNGHGTHVAGTVAALDNSIGVVGVAPSADLYAVKVLGANGRGSVSGIAQGLEWAAANNMHIANMSLGTDAPSSTLERAVNYATSRDVLVIAATGNNGSGSVGYPARYANAMAVGATDQNNRRANFSQYGTGIDIVAPGVNVQSTYPGNRYVSMNGTSMATPHVAGAAALVKQRYPSWNATQIRDHLKNTATNLGNSSQFGSGLVNAEAATR

SEQ ID NO: 57 - DNA, 807 bp, artificial sequence
  B. gibsonii-clade subtilisin
caacaaacagtgccatggggaattactcgtgtgcaagccccagctgttcataaccgtggaattacaggttctggtgtaaaagttgctatcctcgattcaggtatttccacacatgaagacttaaatattcgtggtggcgttagctttgtaccaggggaaccaacgtatgctgatttaaatgggcatggcacgcatgtggctgggacggtagctgctttagacaattcgattggcgttgttggcgtagcaccgtcagcggatctatacgctgttaaagtattaggggcgaatggtagaggttcggtcagcgggattgcccaaggattggaatgggcagcacaaaataacatgcacgttgctaatatgagtttaggaacagatgcaccaagttctacacttgagcgtgctgttaattatgcgacttctagagatgttcttgttattgcggcaactgggaataacggttctggctcagtaggctatccggcccgttatgcgaacgcaatggcagtcggagctactgaccaaaacaacagacgcgccaacttttcacagtatggcacggggattgacattgtcgcaccaggtgtaaacgtgcagagcacatacccaggtaaccgttatgtgagcatgaacggtacatcgatggctactcctcatgttgcaggtgcagcagcccttgttaaacaacgctatccatcttggaatgcgactcaaatccgcgaccatctaaagaatacggcaacgaatttaggaaactcttcacaatatggaagcggacttgtcaatgcagaagcggcaacacgc

SEQ ID NO: 58 - protein, 269 aa, artificial sequence
  B. gibsonii-clade subtilisin
QQTVPWGITRVQAPAVHNRGITGSGVKVAILDSGISTHEDLNIRGGVSFVPGEPTYADLNGHGTHVAGTVAALDNSIGVVGVAPSADLYAVKVLGANGRGSVSGIAQGLEWAAQNNMHVANMSLGTDAPSSTLERAVNYATSRDVLVIAATGNNGSGSVGYPARYANAMAVGATDQNNRRANFSQYGTGIDIVAPGVNVQSTYPGNRYVSMNGTSMATPHVAGAAALVKQRYPSWNATQIRDHLKNTATNLGNSSQYGSGLVNAEAATR

SEQ ID NO: 59 - DNA, 807 bp, artificial sequence
  B. gibsonii-clade subtilisin
caacaaacagtgccatggggaattactcgtgtgcaagccccagctgttcataaccgtggaattacaggttctggtgtaaaagttgctatcctcgattcaggtatttccacacatgaagacttaaatgttcgtggtggcgttagctttgtaccaggggaaccaacgactgctgatttaaatgggcatggcacgcatgtggctgggacggtagctgctttaaacaattcgattggcgttgttggcgtagcaccgtcagcggatctatacgctgttaaagtattaggggcgaatggtagaggttcggtcagcgggattgcccaaggattggaatgggcagcagcaaataacatgcacattgctaatatgagtttaggaacagatgcaccaagttctacacttgagcgtgctgttaattatgcgacttctagagatgttcttgttattgcggcaactgggaataacggttctggctcagtaggctatccggcccgttatgcgaacgcaatggcagtcggagctactgaccaaaacaacagacgcgccaacttttcacagtatggcacggggattgacattgtcgcaccaggtgtaaacgtgcagagcacatacccaggtaaccgttatgtgagcatgaacggtacatcgatggctactcctcatgttgcaggtgcagcagcccttgttaaacaacgctatccatcttggaatgcgactcaaatccgcgaccatctaaagaatacggcaacgaatttaggaaactcttcacaatttggaagcggacttgtcaatgcagaagcggcaacacgc

SEQ ID NO: 60 - protein, 269 aa, artificial sequence
  B. gibsonii-clade subtilisin
QQTVPWGITRVQAPAVHNRGITGSGVKVAILDSGISTHEDLNVRGGVSFVPGEPTTADLNGHGTHVAGTVAALNNSIGVVGVAPSADLYAVKVLGANGRGSVSGIAQGLEWAAANNMHIANMSLGTDAPSSTLERAVNYATSRDVLVIAATGNNGSGSVGYPARYANAMAVGATDQNNRRANFSQYGTGIDIVAPGVNVQSTYPGNRYVSMNGTSMATPHVAGAAALVKQRYPSWNATQIRDHLKNTATNLGNSSQFGSGLVNAEAATR

SEQ ID NO: 61 - DNA, 807 bp, artificial sequence
  B. gibsonii-clade subtilisin
caacaaacagtgccatggggaattactcgtgtgcaagccccagctgttcataaccgtggaattacaggttctggtgtaagagttgctatcctcgattcaggtatttccacacatgaagacttaaatgttcgtggtggcgttagctttgtaccaggggaaccaacgtatgctgatttaaatgggcatggcacgcatgtggctgggacggtagctgctttaaacaattcgattggcgttgttggcgtagcaccgtcagcggatctatacgctgttaaagtattaggggcgaatggtagaggttcggtcagcgggattgcccaaggattggaatgggcagcagcaaataacatgcacattgctaatatgagtttaggaacagatgcaccaagttctacacttgagcgtgctgttaattatgcgacttctgcagatgttcttgttattgcggcaactgggaataacggttctggctcagtaggctatccggcccgttatgcgaacgcaatggcagtcggagctactgaccaaaacaacagacgcgccaacttttcacagtatggcacggggattgacattgtcgcaccaggtgtaaacgtgcagagcacatacccaggtaaccgttatgtgagcatgaacggtacatcgatggctactcctcatgttgcaggtgcagcagcccttgttaaacaacgctatccatcttggaatgcgactcaaatccgcaatcatctaaagaatacggcaacgaatttaggaaactcttcacaatttggaagcggacttgtcaatgcagaagcggcaacacgc

SEQ ID NO: 62 - protein, 269 aa, artificial sequence
  B. gibsonii-clade subtilisin
QQTVPWGITRVQAPAVHNRGITGSGVRVAILDSGISTHEDLNVRGGVSFVPGEPTYADLNGHGTHVAGTVAALNNSIGVVGVAPSADLYAVKVLGANGRGSVSGIAQGLEWAAANNMHIANMSLGTDAPSSTLERAVNYATSADVLVIAATGNNGSGSVGYPARYANAMAVGATDQNNRRANFSQYGTGIDIVAPGVNVQSTYPGNRYVSMNGTSMATPHVAGAAALVKQRYPSWNATQIRNHLKNTATNLGNSSQFGSGLVNAEAATR

SEQ ID NO: 63 - DNA, 807 bp, artificial sequence
  B. gibsonii-clade subtilisin
caacaaacaattccatggggaattagccgtgtgcaagccccagctgttcataaccgtggaattacaggttctggtgtaagagttgctatcctcgattcaggtatttccacacatgaagacttaaatgttcgtggtggcgttagctttgtaccaggggaaccaacgactgctgatttaaatgggcatggcacgcatgtggctgggacggtagctgctttaaacaattcgattggcgttgttggcgtagcaccgtcagcggatctatacgctgttaaagtattaggggcgaatggtagaggttcggtcagcgggattgcccaaggattggaatgggcagcagcaaataacatgcacattgctaatatgagtttaggaagcgatgcaccaagttctacacttgagcgtgctgttaattatgcgacttctagagatgttcttgttattgcggcaactgggaataacggttctggctcagtaggctatccggcccgttatgcgaacgcaatggcagtcggagctactgaccaaaacaacagacgcgccaacttttcacagtatggcacggggattgacattgtcgcaccaggtgtaaacgtgcagagcacatacccaggtaaccgttatgtgagcatgaacggtacatcgatggctactcctcatgttgcaggtgttgcagcccttgttaaacaacgctatccatcttggaatgcgactcaaatccgcaatcatctactgaatacggcaacgaatttaggaaactctaaccaatttggaagcggacttgtcaatgcagaagcggcaacacgc

SEQ ID NO: 64 - protein, 269 aa, artificial sequence
  B. gibsonii-clade subtilisin
QQTIPWGISRVQAPAVHNRGITGSGVRVAILDSGISTHEDLNVRGGVSFVPGEPTTADLNGHGTHVAGTVAALNNSIGVVGVAPSADLYAVKVLGANGRGSVSGIAQGLEWAAANNMHIANMSLGSDAPSSTLERAVNYATSRDVLVIAATGNNGSGSVGYPARYANAMAVGATDQNNRRANFSQYGTGIDIVAPGVNVQSTYPGNRYVSMNGTSMATPHVAGVAALVKQRYPSWNATQIRNHLLNTATNLGNSNQFGSGLVNAEAATR

SEQ ID NO: 65 - DNA, 807 bp, artificial sequence
  B. gibsonii-clade subtilisin
caacaaacagtgccatggggaattactcgtgtgcaagccccagctgttcataaccgtggaattacaggttctggtgtaagagttgctatcctcgattcaggtatttccacacatgaagacttaaatgttcgtggtggcgttagctttgtaccaggggaaccaacgtatgctgatttaaatgggcatggcacgcatgtggctgggacggtagctgctttaaacaattcgattggcgttgttggcgtagcaccgtcagcggatctatacgctgttaaagtattaggggcgaatggtagaggttcggtcagcgggattgcccaaggattggaatgggcagcacaaaataacatgcacattgctaatatgagtttaggaacagatgcaccaagttctacacttgagcgtgctgttaattatgcgacttctagagatgttcttgttattgcggcaactgggaataacggttctggctcagtaggctatccggcccgttatgcgaacgcaatggcagtcggagctactgaccaaaacaacagacgcgccaacttttcacagtatggcacggggattgacattgtcgcaccaggtgtaaacgtgcagagcacatacccaggtaaccgttatgtgagcatgaacggtacatcgatggctactcctcatgttgcaggtgcagcagcccttgttaaacaacgctatccatcttggaatgcgactcaaatccgcgaccatctaaagaatacggcaacgaatttaggaaactcttcacaatttggaagcggacttgtcaatgcagaagcggcaacacgc

SEQ ID NO: 66 - protein, 269 aa, artificial sequence
  B. gibsonii-clade subtilisin
QQTVPWGITRVQAPAVHNRGITGSGVRVAILDSGISTHEDLNVRGGVSFVPGEPTYADLNGHGTHVAGTVAALNNSIGVVGVAPSADLYAVKVLGANGRGSVSGIAQGLEWAAQNNMHIANMSLGTDAPSSTLERAVNYATSRDVLVIAATGNNGSGSVGYPARYANAMAVGATDQNNRRANFSQYGTGIDIVAPGVNVQSTYPGNRYVSMNGTSMATPHVAGAAALVKQRYPSWNATQIRDHLKNTATNLGNSSQFGSGLVNAEAATR

SEQ ID NO: 67 - DNA, 807 bp, artificial sequence
  B. gibsonii-clade subtilisin
caacaaacagtgccatggggaattactcgtgtgcaagccccagctgttcataaccgtggaattacaggttctggtgtaagagttgctatcctcgattcaggtatttccacacatgaagacttaaatgttcgtggtggcgttagctttgtaccaggggaaccaacgtatgctgatttaaatgggcatggcacgcatgtggctgggacggtagctgctttaaacaattcgattggcgttgttggcgtagcaccgtcagcggatctatacgctgttaaagtattaggggcgaatggtagaggttcggtcagcgggattgcccaaggattggaatgggcagcacaaaataacatgcacgttgctaatatgagtttaggaacagatgcaccaagttctacacttgagcgtgctgttaattatgcgacttctagagatgttcttgttattgcggcaactgggaataacggttctggctcagtaggctatccggcccgttatgcgaacgcaatggcagtcggagctactgaccaaaacaacagacgcgccaacttttcacagtatggcacggggattgacattgtcgcaccaggtgtaaacgtgcagagcacatacccaggtaaccgttatgtgagcatgaacggtacatcgatggctactcctcatgttgcaggtgcagcagcccttgttaaacaacgctatccatcttggaatgcgactcaaatccgcgaccatctaaagaatacggcaacgaatttaggaaactcttcacaatttggaagcggacttgtcaatgcagaagcggcaacacgc

SEQ ID NO: 68 - protein, 269 aa, artificial sequence
  B. gibsonii-clade subtilisin
QQTVPWGITRVQAPAVHNRGITGSGVRVAILDSGISTHEDLNVRGGVSFVPGEPTYADLNGHGTHVAGTVAALNNSIGVVGVAPSADLYAVKVLGANGRGSVSGIAQGLEWAAQNNMHVANMSLGTDAPSSTLERAVNYATSRDVLVIAATGNNGSGSVGYPARYANAMAVGATDQNNRRANFSQYGTGIDIVAPGVNVQSTYPGNRYVSMNGTSMATPHVAGAAALVKQRYPSWNATQIRDHLKNTATNLGNSSQFGSGLVNAEAATR

SEQ ID NO: 69 - DNA, 807 bp, artificial sequence
  B. gibsonii-clade subtilisin
caacaaacagtgccatggggaattactcgtgtgcaagccccagctgttcataaccgtggaattacaggttctggtgtaagagttgctatcctcgattcaggtatttccacacatgaagacttaaatgttcgtggtggcgttagctttgtaccaggggaaccaacgactgctgatttaaatgggcatggcacgcatgtggctgggacggtagctgctttagacaattcgattggcgttgttggcgtagcaccgtcagcggatctatacgctgttaaagtattaggggcgaatggtagaggttcgattagcgggattgcccaaggattggaatgggcagcagcaaataacatgcacattgctaatatgagtttaggaagcgatgcaccaagttctacacttgagcgtgctgttaattatgcgacttctcaagatgttcttgttattgcggcaactgggaataacggttctggcacagtaggctatccggcccgttatgcgaacgcaatggcagtcggagctactgaccaaaacaacagacgcgccaacttttcacagtatggcacggggattgacattgtcgcaccaggtgtaaacgtgcagagcacatacccaggtaaccgttatgtgagcatgaacggtacatcgatggctactcctcatgttgcaggtgttgcagcccttgttaaacaacgctatccatcttggaatgcgactcaaatccgcaatcatctaaagaatacggcaacgaatttaggaaactctaaccaatttggaagcggacttgtcaatgcagaagcggcaacacgc

SEQ ID NO: 70 - protein, 269 aa, artificial sequence
  B. gibsonii-clade subtilisin
QQTVPWGITRVQAPAVHNRGITGSGVRVAILDSGISTHEDLNVRGGVSFVPGEPTTADLNGHGTHVAGTVAALDNSIGVVGVAPSADLYAVKVLGANGRGSISGIAQGLEWAAANNMHIANMSLGSDAPSSTLERAVNYATSQDVLVIAATGNNGSGTVGYPARYANAMAVGATDQNNRRANFSQYGTGIDIVAPGVNVQSTYPGNRYVSMNGTSMATPHVAGVAALVKQRYPSWNATQIRNHLKNTATNLGNSNQFGSGLVNAEAATR

SEQ ID NO: 71 - protein, 34 aa, artificial sequence
  motif
  MISC_FEATURE (1)..(34): where the initial D is the active site Aspartic acid residue, the penultimate H is the active site Histidine, and X is any amino acid, and where the amino acid positions of the variant are numbered by correspondence with the amino acid sequence of SEQ ID
  MISC_FEATURE (2)..(2): Xaa is any amino acid
  MISC_FEATURE (5)..(6): Xaa is any amino acid
  MISC_FEATURE (11)..(13): Xaa is any amino acid
  MISC_FEATURE (18)..(22): Xaa is any amino acid
  MISC_FEATURE (30)..(30): Xaa is any amino acid
DXGIXXHSDLXXXGGASXXXXXPTTADLNXHGTH

SEQ ID NO: 72 - protein, 34 aa, artificial sequence
  motif
  MISC_FEATURE (1)..(34): where the initial D is the active site Aspartic acid residue, the penultimate H is the active site Histidine, and X is any amino acid, and where the amino acid positions of the variant are numbered by correspondence with the amino acid sequence of SEQ ID
  MISC_FEATURE (2)..(2): Xaa is any amino acid
  MISC_FEATURE (5)..(6): Xaa is any amino acid
  MISC_FEATURE (11)..(13): Xaa is any amino acid
  MISC_FEATURE (18)..(23): Xaa is any amino acid
  MISC_FEATURE (29)..(30): Xaa is any amino acid
DXGIXXHSDLXXXGGASXXXXXXTTADLXXHGTH

SEQ ID NO: 73 - skipped

SEQ ID NO: 74 - protein, 275 aa, B. amyloliquefaciens [sequence omitted]

SEQ ID NO: 75 - protein, 275 aa, G. stearothermophilus
AQSVPYGVSQIKAPALHSQGFTGSNVKVAVIDSGIDSSHPDLKVAGGASMVPSETNPFQDNNSHGTHVAGTVAALNNSVGVLGVAPSASLYAVKVLGADGSGQYSWIINGIEWAIAYNMDVINMSLGGPSGSAALKAAVDKAVASGIVVVAAAGNEGTSGSSSTVGYPGKYPSVIAVGAVNSSNQRASFSSVGSELDVMAPGVSIQSTLPGNKYGAYNGTSMASPHVAGAAALILSKHPNWTNTQVRSSLENTTTKLGDAFYYGKGLINVQAAAQ

SEQ ID NO: 76 - protein, 275 aa, B. subtilis
AQSVPYGISQIKAPALHSQGYTGSNVKVAVIDSGIDSSHPDLNVRGGASFVPSETNPYQDGSSHGTHVAGTVAALNNTIGVLGVAPSASLYAVKVLDSTGSGQYSWIINGIEWAISNNMDVINMSLGGPTGSTALKTVVDKAVASGIVVVAAAGNEGSSGSTSTVGYPAKYPSTIAVGAVNSSNQRASFSSAGSELDVMAPGVSIQSTLPGGTYGSYNGTSMATPHVAGAAALILSKHPTWSNAQVRDRLESTATNLGSSFYYGKGLINVQAAAQ

SEQ ID NO: 77 - protein, 275 aa, B. atrophaeus
AQSVPYGISQIKAPAVHSQGYTGSNVKVAVIDSGIDSSHPDLKVSGGASFVPSEPNPFQDGNSHGTHVAGTVAALNNSVGVLGVAPSASLYAVKVLSSSGSGDYSWIINGIEWAISNNMDVINMSLGGPQGSTALKAVVDKAVSQGIVVVAAAGNSGSSGSTSTVGYPAKYPSVIAVGAVDSNNQRASFSSAGSELDVMAPGVSIQSTLPGSSYGSYNGTSMASPHVAGAAALVLSKHPNWTNSQVRNSLESTATNLGNSFYYGKGLINVQAAAQ

SEQ ID NO: 78 - protein, 275 aa, B. circulans
AQTVPYGIPQIKAPAVHAQGYKGANVKVAVLDTGIHAAHPDLNVAGGASFVPSEPNATQDFQSHGTHVAGTIAALDNTIGVLGVAPSASLYAVKVLDRNGDGQYSWIISGIEWAVANNMDVINMSLGGPNGSTALKNAVDTANNRGVVVVAAAGNSGSTGSTSTVGYPAKYDSTIAVANVNSSNVRNSSSSAGPELDVSAPGTSILSTVPSRGYTSYTGTSMASPHVAGAAALILSKNPNLSNSQVRQRLENTATPLGNSFYYGKGLINVQAASN

SEQ ID NO: 79 - protein, 275 aa, B. pumilus
AQTVPYGIPQIKAPAVHAQGYKGANVKVAVLDTGIHAAHPDLNVAGGASFVPSEPNATQDFQSHGTHVAGTIAALDNTIGVLGVAPSASLYAVKVLDRNGDGQYSWIISGIEWAVANNMDVINMSLGGASGSTALKNAVDTANNRGVVVVAAAGNSGSSGSRSTVGYPAKYESTIAVANVNSNNVRNSSSSAGPELDVSAPGTSILSTVPSSGYTSYTGTSMASPHVAGAAALILSKNPNLTNSQVRQRLENTATPLGDSFYYGKGLINVQAASN

SEQ ID NO: 80 - protein, 274 aa, B. licheniformis
AQTVPYGIPLIKADKVQAQGFKGANVKVAVLDTGIQASHPDLNVVGGASFVAGEAYNTDGNGHGTHVAGTVAALDNTTGVLGVAPSVSLYAVKVLNSSGSGSYSGIVSGIEWATTNGMDVINMSLGGASGSTAMKQAVDNAYARGVVVVAAAGNSGSSGNTNTIGYPAKYDSVIAVGAVDSNSNRASFSSVGAELEVMAPGAGVYSTYPTNTYATLNGTSMASPHVAGAAALILSKHPNLSASQVRNRLSSTATYLGSSFYYGKGLINVEAAAQ

SEQ ID NO: 81 - protein, 275 aa, unknown
  Bacillus sp.
AQTTPWGVTHINAHRAHSSGVTGSGVKVAILDTGIHASHPDLNVRGGASFISGESNPYIDSNGHGTHVAGTVAALNNTVGVLGVAYNAELYAVKVLSASGSGTLSGIAQGVEWSIANKMDVINMSLGGSSGSTALQRAVDNAYRNNIVVVAAAGNSGAQGNRNTIGYPARYSSVIAVGAVDSNNNRASFSSVGSELEVMAPGVSILSTVPGSSYASYNGTSMASPHVAGAAALLKAKYPNWSAAQIRNKLNSTTTYLGSSFYYGNGVINVERALQ

SEQ ID NO: 82 - protein, 275 aa, unknown
  bacillus sp.
AQTVPWGIPHIKADKAHAAGVTGSGVKVAILDTGIDANHADLNVKGGASFVSGEPNALQDGNGHGTHVAGTVAALNNTTGVLGVAYNADLYAVKVLSASGSGTLSGIAQGIEWSISNGMNVINMSLGGSSGSTALQQACNNAYNRGIVVIAAAGNSGSSGNRNTMGYPARYSSVIAVGAVSSNNTRASFSSVGSELEVMAPGVNILSTTPGNNYASFNGTSMAAPHVAGAAALIKAKYPSMTNVQIRERLKNTATNLGDPFFYGKGVINVESALQ

SEQ ID NO: 83 - protein, 269 aa, unknown
  bacillus sp.
SQTVPWGISFINTQQAHNRGIFGNGARVAVLDTGIASHPDLRIAGGASFISSEPSYHDNNGHGTHVAGTIAALNNSIGVLGVAPSADLYAVKVLDRNGSGSLASVAQGIEWAINNNMHIINMSLGSTSGSSTLELAVNRANNAGILLVGAAGNTGRQGVNYPARYSGVMAVAAVDQNGQRASFSTYGPEIEISAPGVNVNSTYTGNRYVSLSGTSMATPHVAGVAALVKSRYPSYTNNQIRQRINQTATYLGSPSLYGNGLVHAGRATQ

SEQ ID NO: 84 - protein, 269 aa, B. lentus
AQSVPWGISRVQAPAAHNRGLTGSGVKVAVLDTGISTHPDLNIRGGASFVPGEPSTQDGNGHGTHVAGTIAALNNSIGVLGVAPSAELYAVKVLGASGSGSVSSIAQGLEWAGNNGMHVANLSLGSPSPSATLEQAVNSATSRGVLVVAASGNSGAGSISYPARYANAMAVGATDQNNNRASFSQYGAGLDIVAPGVNVQSTYPGSTYASLNGTSMATPHVAGAAALVKQKNPSWSNVQIRNHLKNTATSLGSTNLYGSGLVNAEAATR

SEQ ID NO: 85 - protein, 269 aa, B. gibsonii
QQTVPWGITRVQAPAVHNRGITGSGVRVAILDSGISAHSDLNIRGGASFVPGEPTTADLNGHGTHVAGTVAALNNSIGVIGVAPNAELYAVKVLGANGSGSVSGIAQGLEWAATNNMHIANMSLGSDFPSSTLERAVNYATSRDVLVIAATGNNGSGSVGYPARYANAMAVGATDQNNRRANFSQYGTGIDIVAPGVNVQSTYPGNRYVSMNGTSMATPHVAGAAALVKQRYPSWNATQIRNHLKNTATNLGNSSQFGSGLVNAEAATR

SEQ ID NO: 86 - protein, 269 aa, B. gibsonii
QQTVPWGITRVQAPAVHNRGVTGSGVRVAILDSGISTHSDLTIRGGASFVPGEPTTADLNGHGTHVAGTVAALNNSIGVIGVAPSADLYAVKVLGANGRGSVSGIAQGLEWAAANNMHIANMSLGSDAPSTTLERAVNYATSQGVLVIAATGNNGSGSVGYPARYANAMAVGATDQNNRRANFSQYGTGIDIVAPGVNVQSTYPGNRYASLNGTSMATPHVAGAAALVKQRYPSWNATQIRNHLKNTATNLGNSSQFGSGLVNAEAATR

SEQ ID NO: 87 - protein, 269 aa, B. gibsonii
QQTVPWGITRVQAPAVHNRGITGSGVRVAILDSGISAHSDLNIRGGASFVPGEPTTADLNGHGTHVAGTVAALNNSIGVIGVAPNADLYAVKVLGANGSGSVSGIAQGLEWAATNNMHIANMSLGSDFPSSTLERAVNYATSRDVLVIAATGNNGSGSVGYPARYANAMAVGATDQNNRRANFSQYGTGIDIVAPGVNVQSTYPGNRYVSMNGTSMATPHVAGAAALVKQRYPSWNATQIRNHLKNTATNLGNSSQFGSGLVNAEAATR

SEQ ID NO: 88 - protein, 269 aa, B. gibsonii
QQTVPWGITRVQAPAVHNRGVTGSGVRVAILDSGISTHSDLTIRGGASFVPGEPTTADLNGHGTHVAGTVAALNNSIGVIGVAPSADLYAVKVLGANGRGSVSGIAQGLEWAAANNMHIANMSLGSDAPSTTLERAVNYATSQGVLVIAATGNNGSGSVGYPARYANAMAVGATDQNNRRANFSQYGTGIDIVAPGVNVQSTYPGNRYVSMNGTSMATPHVAGAAALVKQRYPSWNATQIRNHLKNTATNLGNSSQFGSGLVNAEAATR

SEQ ID NO: 89 - protein, 269 aa, B. gibsonii
QQTVPWGITRVQAPAVHNRGVTGSGVRVAILDSGISTHSDLTIRGGASFVPGEPTTADLNGHGTHVAGTVAALNNSIGVIGVAPSADLYAVKVLGANGRGSVSGIAQGLEWAAANNMHIANMSLGSDAPSTTLERAVNYATSQGVLVIAATGNNGSGSVGYPARYANAMAVGATDQNNRRANFSQYGSGIDIVAPGVNVQSTYPGNRYVSMNGTSMATPHVAGAAALVKQRYPSWNATQIRNHLKNTATNLGNSSQFGSGLVNAEAATR

SEQ ID NO: 90 - protein, 269 aa, B. gibsonii
QQTVPWGITRVQAPAVHNRGVTGSGVRVAILDSGISTHSDLTIRGGASFVPGEPTTADLNGHGTHVAGTVAALNNSIGVIGVAPSADLYAVKVLGANGRGSVSGIAQGLEWAAANNMHIANMSLGSDAPSITLERAVNYATSQGVLVIAATGNNGSGSVGYPARYANAMAVGATDQNNRRANFSQYGTGIDIVAPGVNVQSTYPGNRYASLNGTSMATPHVAGAAALVKQRYPSWNATQIRNHLKNTATNLGNSSQFGSGLVNAEAATR

SEQ ID NO: 91 - protein, 269 aa, B. gibsonii
QQTVPWGITRVQAPTVHNRGITGSGVKVAILDTGIAQHSDLTIRGGASFVPGESTTADLNGHGTHVAGTVAALNNSIGVIGVAPSADLYAVKVLGANGRGSVSGIAQGLEWAATNNMHIANMSLGSDAPSTTLERAVNYATSRGVLVIAATGNNGTGSIGYPARYANAMAVGATDQNNRRASFSQYGTGIDIVAPGVGIQSTYLNNSYASMPGTSMATPHVAGVAALVKQKNPSWNATQIRNHLKNTATNLGNSSQFGSGLVNADAATR

SEQ ID NO: 92 - protein, 269 aa, B. gibsonii
QQTVPWGITRVQAPAVHNRGVTGSGVRVAILDSGISQHSDLTIRGGASFIPGEPTTADLNGHGTHVAGTVAALNNSIGVIGVAPSADLYAVKVLGANGRGSVSGIAQGLEWAAANNMHIANMSLGADAPSSTLERAVNYATSQGVLVIAATGNNGSGSVGYPARYANAMAVGATDQNNRRANFSQYGTGIDIVAPGVNVQSTYPGNRYASLNGTSMATPHVAGAAALVKQRNPSWNATQIRNHLKNTATNLGNSSQFGSGLVNAEAATR

SEQ ID NO: 93 - protein, 269 aa, B. gibsonii
QQTVPWGITRVQAPAVHNRGVTGSGVRVAILDSGISQHSDLTIRGGASFVPGEPTTEDLNGHGTHVAGTVAALNNSFGVIGVAPSADLYAVKVLGAGGRGSVSGIAQGLEWAAANNMHIANMSLGADAPSSTLERAVNYATSRGVLVIAATGNNGSGSVGYPARYANAMAVGATDQNNRRANFSQYGTGIDIVAPGVNVQSTYPGNRYASLNGTSMATPHVAGVAALVKQRNPSWNATQIRNHLKNTATNLGNSSQFGSGLVNAEAAIR

SEQ ID NO: 94 - protein, 269 aa, artificial sequence
  B. gibsonii-clade subtilisin
QQTVPWGITRVQAPAVHNRGVTGSGVRVAILDSGISAHSDLNIRGGASFVPGEPTTADLNGHGTHVAGTVAALNNSIGVVGVAPSADLYAVKVLGANGSGSVSGIAQGLEWAATNNIHIANMSLGSDAPSTTLERAVNYATSQGVLVIAATGNNGSGSVGYPARYANAMAVGATDQNNRRANFSQYGTGIDIVAPGVNVQSTYPGNRYVSMNGTSMATPHVAGVAALVKQRYPSWNATQIRNHLKNTATNLGNSSQFGSGLVNAEAATR

SEQ ID NO: 95 - protein, 269 aa, artificial sequence
  B. gibsonii-clade subtilisin
QQTVPWGITRVQAPAVHNRGITGSGVRVAILDSGISAHSDLTIRGGASFVPGEPTTADLNGHGTHVAGTVAALNNSIGVVGVAPSADLYAVKVLGANGSGSVSGIAQGLEWAAANNMHIANMSLGSDAPSSTLERAVNYATSQGVLVIAATGNNGSGTISYPARYANAMAVGATDQNNRRANFSQYGTGIDIVAPGVGVQSTYPGNRYVSMNGTSMATPHVAGAAALVKQRYPSWNATQIRNHLKNTATNLGNSSQFGSGLVNAEAATR

SEQ ID NO: 96 - protein, 269 aa, artificial sequence
  B. gibsonii-clade subtilisin
AQTVPWGITRVQAPAVHNRGITGSGVRVAILDSGISAHSDLNIRGGASFVPGEPTTADLNGHGTHVAGTVAALNNSIGVVGVAPNAELYAVKVLGANGSGSVSGIAQGLEWAATNNMHIANMSLGSDAPSTTLERAVNYATSAGVLVIAATGNNGSGSVGYPARYANALAVGATDQNNRRANFSQYGTGLDIVAPGVNVQSTYPGNRYVSMNGTSMATPHVAGAAALVKQRYPSWNATQIRNHLKNTATNLGNTNLYGSGLVNAEAATR

SEQ ID NO: 97 - protein, 269 aa, artificial sequence
  B. gibsonii-clade subtilisin
QQTVPWGITRVQAPAVHNRGITGSGVRVAILDSGISAHSDLNIRGGASFVPGEPTTADLNGHGTHVAGTVAALDNSIGVVGVAPSADLYAVKVLGANGSGSVSGIAQGLEWAATNNMHIANMSLGSDFPSSTLERAVNYATSRDVLVIAATGNNGSGTVGYPARYANAMAVGATDQNNRRANFSQYGTGIDIVAPGVNVQSTYPGNRYVSMNGTSMATPHVAGAAALVKQRYPSWNATQIRDHLKNTATNLGNSSQFGSGLVNAEAATR

SEQ ID NO: 98 - protein, 269 aa, artificial sequence
  B. gibsonii-clade subtilisin
QQTVPWGITRVQAPAVHNRGITGSGVRVAILDSGISAHSDLNIRGGASFVPGEPTTADLNGHGTHVAGTVAALDNSIGVVGVAPSADLYAVKVLGANGRGSISGIAQGLEWAATNNMHIANMSLGSDFPSSTLERAVNYATSRDVLVIAATGNNGSGTIGYPARYANAMAVGATDQNNRRANFSQYGTGIDIVAPGVNVQSTYPGNRYVSMNGTSMATPHVAGAAALVKQRYPSWNATQIRDHLKNTATNLGNSSQYGSGLVNAEAATR

SEQ ID NO: 99 - protein, 269 aa, artificial sequence
  B. gibsonii-clade subtilisin
QQTVPWGITRVQAPAVHNRGITGSGVRVAILDSGISAHSDLNIRGGASFVPGEPTTADLNGHGTHVAGTVAALNNSIGVIGVAPSADLYAVKVLGANGRGSISGIAQGLEWAAQNNMHIANMSLGSDFPSSTLERAVNYATSRDVLVIAATGNNGSGTISYPARYANAMAVGATDQNNRRANFSQYGTGIDIVAPGVNVQSTYPGNRYVSMSGTSMATPHVAGAAALVKQRYPSWNATQIRDHLKNTATNLGNSSQYGSGLVNAEAATR

SEQ ID NO: 100 - protein, 269 aa, artificial sequence
  B. gibsonii-clade subtilisin
QQTVPWGITRVQAPAVHNRGITGSGVRVAILDSGISAHSDLNIRGGASFVPGEPTTADLNGHGTHVAGTVAALDNSIGVVGVAPSADLYAVKVLGANGRGSISGIAQGLEWAATNNMHIANMSLGTDAPSSTLERAVNYATSADVLVIAATGNNGSGSVGYPARYANAMAVGATDQNNRRANFSQYGTGLDIVAPGVNVQSTYPGNRYVSMNGTSMATPHVAGAAALVKQRYPSWNATQIRDHLKNTATNLGNSSQYGSGLVNAEAATR

SEQ ID NO: 101 - protein, 269 aa, artificial sequence
  B. gibsonii-clade subtilisin
QQTVPWGITRVQAPAVHNRGITGSGVRVAILDSGISAHSDLNIRGGASFVPGEPTTADLNGHGTHVAGTVAALDNSIGVVGVAPSADLYAVKVLGANGRGSISGIAQGLEWAAQNNMHIANMSLGSDFPSSTLERAVNYATSADVLVIAATGNNGSGSVGYPARYANAMAVGATDQNNRRANFSQYGTGLDIVAPGVNVQSTYPGNRYVSMNGTSMATPHVAGAAALVKQRYPSWNATQIRDHLKNTATNLGNSSQYGSGLVNAEAATR

SEQ ID NO: 102 - protein, 269 aa, artificial sequence
  B. gibsonii-clade subtilisin
QQTVPWGITRVQAPAVHNRGITGSGVRVAILDSGISAHSDLNIRGGASFVPGEPTTADLNGHGTHVAGTVAALDNSIGVVGVAPSADLYAVKVLGANGRGSISGIAQGLEWAATNNMHIANMSLGSDFPSSTLERAVNYATSRDVLVIAATGNNGSGSVGYPARYANAMAVGATDQNNRRANFSQYGTGLDIVAPGVNVQSTYPGNRYVSMNGTSMATPHVAGAAALVKQRYPSWNATQIRDHLKNTATNLGNSSQYGSGLVNAEAATR

SEQ ID NO: 103 - protein, 269 aa, artificial sequence
  B. gibsonii-clade subtilisin
QQTVPWGITRVQAPAVHNRGITGSGVRVAILDSGISAHSDLNIRGGASFVPGEPTTADLNGHGTHVAGTVAALDNSIGVIGVAPSADLYAVKVLGANGRGSISGIAQGLEWAATNNMHIANMSLGTDAPSSTLERAVNYATSRDVLVIAATGNNGSGSVGYPARYANAMAVGATDQNNRRANFSQYGTGLDIVAPGVNVQSTYPGNRYVSMNGTSMATPHVAGAAALVKQRYPSWNATQIRDHLKNTATNLGNSSQYGSGLVNAEAATR

SEQ ID NO: 104 - protein, 269 aa, artificial sequence
  B. gibsonii-clade subtilisin
QQTVPWGITRVQAPAVHNRGITGSGVRVAILDSGISAHSDLNIRGGASFVPGEPTTADLNGHGTHVAGTVAALDNSIGVIGVAPNAELYAVKVLGANGRGSISGIAQGLEWAATNNMHIANMSLGTDAPSSTLERAVNYATSADVLVIAATGNNGSGTVGYPARYANAMAVGATDQNNRRANFSQYGTGIDIVAPGVNVQSTYPGNRYVSMSGTSMATPHVAGAAALVKQRYPSWNATQIRNHLKNTATNLGNSSQFGSGLVNAEAATR

SEQ ID NO: 105 - protein, 269 aa, artificial sequence
  B. gibsonii-clade subtilisin
QQTVPWGITRVQAPAVHNRGITGSGVRVAILDSGISAHSDLNIRGGASFVPGEPTTADLNGHGTHVAGTVAALDNSIGVVGVAPNAELYAVKVLGANGRGSISGIAQGLEWAAQNNMHVANMSLGTDAPSSTLERAVNYATSRDVLVIAATGNNGSGTVSYPARYANAMAVGATDQNNRRANFSQYGTGIDIVAPGVNVQSTYPGNRYVSMSGTSMATPHVAGAAALVKQRYPSWNATQIRNHLKNTATNLGNSSQYGSGLVNAEAATR

SEQ ID NO: 106 - protein, 269 aa, artificial sequence
  B. gibsonii-clade subtilisin
QQTVPWGITRVQAPAVHNRGITGSGVKVAILDSGISAHSDLNIRGGASFVPGEPTTADLNGHGTHVAGTVAALNNSIGVIGVAPNAELYAVKVLGANGRGSISGIAQGLEWAAQNNMHVANMSLGTDAPSSTLERAVNYATSRDVLVIAATGNNGSGTISYPARYANAMAVGATDQNNRRANFSQYGAGIDIVAPGVNVQSTYPGNRYVSMNGTSMATPHVAGAAALVKQRYPSWNATQIRDHLKNTATNLGNSSQFGSGLVNAEAATR

SEQ ID NO: 107 - protein, 269 aa, artificial sequence
  B. gibsonii-clade subtilisin
QQTVPWGITRVQAPAVHNRGITGSGVKVAILDSGISAHSDLNIRGGASFVPGEPTTADLNGHGTHVAGTVAALNNSIGVIGVAPNAELYAVKVLGANGRGSISGIAQGLEWAATNNMHIANMSLGTDAPSSTLERAVNYATSADVLVIAATGNNGSGTISYPARYANAMAVGATDQNNRRANFSQYGTGIDIVAPGVNVQSTYPGNRYVSMNGTSMATPHVAGAAALVKQRYPSWNATQIRNHLKNTATNLGNSSQFGSGLVNAEAATR

SEQ ID NO: 108 - protein, 269 aa, artificial sequence
  B. gibsonii-clade subtilisin
QQTVPWGITRVQAPAVHNRGITGSGVKVAILDSGISAHSDLNIRGGASFVPGEPTTADLNGHGTHVAGTVAALDNSIGVIGVAPNAELYAVKVLGANGRGSISGIAQGLEWAATNNMHVANMSLGTDAPSSTLERAVNYATSADVLVIAATGNNGSGSVSYPARYANAMAVGATDQNNRRANFSQYGTGIDIVAPGVNVQSTYPGNRYVSMSGTSMATPHVAGAAALVKQRYPSWNATQIRDHLKNTATNLGNSSQFGSGLVNAEAATR

SEQ ID NO: 109 - protein, 269 aa, artificial sequence
  B. gibsonii-clade subtilisin
QQTVPWGITRVQAPAVHNRGITGSGVKVAILDSGISAHSDLNIRGGASFVPGEPTTADLNGHGTHVAGTVAALDNSIGVIGVAPNAELYAVKVLGANGRGSISGIAQGLEWAAQNNMHIANMSLGTDAPSSTLERAVNYATSRDVLVIAATGNNGSGSVGYPARYANAMAVGATDQNNRRANFSQYGAGLDIVAPGVNVQSTYPGNRYVSMSGTSMATPHVAGAAALVKQRYPSWNATQIRDHLKNTATNLGNSSQFGSGLVNAEAATR

SEQ ID NO: 110 - protein, 269 aa, artificial sequence
  B. gibsonii-clade subtilisin
QQTVPWGITRVQAPAVHNRGITGSGVRVAILDSGISAHSDLNIRGGASFVPGEPTTADLNGHGTHVAGTVAALDNSIGVVGVAPNAELYAVKVLGANGRGSISGIAQGLEWAAQNNMHIANMSLGTDAPSSTLERAVNYATSADVLVIAATGNNGSGSVGYPARYANAMAVGATDQNNRRANFSQYGTGIDIVAPGVNVQSTYPGNRYVSMSGTSMATPHVAGAAALVKQRYPSWNATQIRDHLKNTATNLGNSSQFGSGLVNAEAATR

SEQ ID NO: 111 - protein, 269 aa, artificial sequence
  B. gibsonii-clade subtilisin
QQTVPWGITRVQAPAVHNRGITGSGVRVAILDSGISAHSDLNIRGGASFVPGEPTTADLNGHGTHVAGTVAALNNSIGVIGVAPSADLYAVKVLGANGRGSVSGIAQGLEWAAQNNMHVANMSLGTDAPSSTLERAVNYATSADVLVIAATGNNGSGSVSYPARYANAMAVGATDQNNRRANFSQYGTGIDIVAPGVNVQSTYPGNRYVSMNGTSMATPHVAGAAALVKQRYPSWNATQIRNHLKNTATNLGNSSQYGSGLVNAEAATR

SEQ ID NO: 112 - protein, 269 aa, artificial sequence
  B. gibsonii-clade subtilisin
QQTVPWGITRVQAPAVHNRGITGSGVRVAILDSGISAHSDLNIRGGASFVPGEPTTADLNGHGTHVAGTVAALNNSIGVVGVAPSADLYAVKVLGANGRGSISGIAQGLEWAAQNNMHVANMSLGTDAPSSTLERAVNYATSADVLVIAATGNNGSGSVGYPARYANAMAVGATDQNNRRANFSQYGTGIDIVAPGVNVQSTYPGNRYVSMNGTSMATPHVAGAAALVKQRYPSWNATQIRDHLKNTATNLGNSSQFGSGLVNAEAATR

SEQ ID NO: 113 - protein, 269 aa, artificial sequence
  B. gibsonii-clade subtilisin
QQTVPWGITRVQAPAVHNRGITGSGVRVAILDSGISAHSDLNIRGGASFVPGEPTTADLNGHGTHVAGTVAALDNSIGVVGVAPSADLYAVKVLGANGRGSVSGIAQGLEWAAQNNMHIANMSLGTDAPSSTLERAVNYATSADVLVIAATGNNGSGSVGYPARYANAMAVGATDQNNRRANFSQYGTGIDIVAPGVNVQSTYPGNRYVSMNGTSMATPHVAGAAALVKQRYPSWNATQIRDHLKNTATNLGNSSQFGSGLVNAEAATR

SEQ ID NO: 114 - protein, 269 aa, artificial sequence
  B. gibsonii-clade subtilisin
QQTVPWGITRVQAPAVHNRGITGSGVRVAILDSGISAHSDLNIRGGASFVPGEPTTADLNGHGTHVAGTVAALDNSIGVVGVAPSADLYAVKVLGANGRGSISGIAQGLEWAAQNNMHIANMSLGTDAPSSTLERAVNYATSRDVLVIAATGNNGSGSVGYPARYANAMAVGATDQNNRRANFSQYGTGIDIVAPGVNVQSTYPGNRYVSMNGTSMATPHVAGAAALVKQRYPSWNATQIRDHLKNTATNLGNSSQFGSGLVNAEAATR

SEQ ID NO: 115 - protein, 275 aa, artificial sequence
  Consensus sequence Figure 6
  MISC_FEATURE (37)..(37): Xaa can be any amino acid
  MISC_FEATURE (57)..(57): Xaa can be any amino acid
  MISC_FEATURE (82)..(82): Xaa can be any amino acid
  MISC_FEATURE (104)..(104): Xaa can be any amino acid
  MISC_FEATURE (116)..(116): Xaa can be any amino acid
  MISC_FEATURE (128)..(128): Xaa can be any amino acid
  MISC_FEATURE (145)..(146): Xaa can be any amino acid
  MISC_FEATURE (159)..(162): Xaa can be any amino acid
  MISC_FEATURE (248)..(248): Xaa can be any amino acid
QQTVPWGITRVQAPAVHNRGITGSGVRVAILDSGISXAHSDLNIRGGASFVPGEPTXTADLNGHGTHVAGTVAALNNSIGVXGVAPSADLYAVKVLGANGRGSXSGIAQGLEWAAXNNMHIANMSLGXDAPSSTLERAVNYATSXXVLVIAATGNNGSXXXXGSVGYPARYANAMAVGATDQNNRRANFSQYGTGIDIVAPGVNVQSTYPGNRYVSMNGTSMATPHVAGAAALVKQRYPSWNATQIRXHLKNTATNLGNSSQFGSGLVNAEAATR

SEQ ID NO: 116 - protein, 269 aa, artificial sequence
  B. gibsonii-clade subtilisin
QQTVPWGITRVQAPAVHNRGITGSGVRVAILDSGISTHEDLNIRGGASFVPGEPTTADLNGHGTHVAGTVAALNNSIGVIGVAPNAELYAVKVLGANGRGSISGIAQGLEWAAQNNMHIANMSLGTDAPSSTLERAVNYATSADVLVIAATGNNGSGSVGYPARYANAMAVGATDQNNRRANFSQYGTGIDIVAPGVNVQSTYPGNRYVSMSGTSMATPHVAGAAALVKQRYPSWNATQIRDHLKNTATNLGNSSQFGSGLVNAEAATR

SEQ ID NO: 117 - protein, 269 aa, artificial sequence
  B. gibsonii-clade subtilisin
QQTVPWGITRVQAPAVHNRGITGSGVRVAILDSGISTHEDLNIRGGASFVPGEPTTADLNGHGTHVAGTVAALDNSIGVIGVAPNAELYAVKVLGANGRGSISGIAQGLEWAATNNMHIANMSLGTDAPSSTLERAVNYATSADVLVIAATGNNGSGSVGYPARYANAMAVGATDQNNRRANFSQYGTGIDIVAPGVNVQSTYPGNRYVSMSGTSMATPHVAGAAALVKQRYPSWNATQIRDHLKNTATNLGNSSQFGSGLVNAEAATR

SEQ ID NO: 118 - protein, 269 aa, artificial sequence
  B. gibsonii-clade subtilisin
QQTVPWGITRVQAPAVHNRGITGSGVRVAILDSGISTHEDLTIRGGASFVPGEPTTADLNGHGTHVAGTVAALNNSIGVIGVAPNAELYAVKVLGANGRGSISGIAQGLEWAAQNNMHIANMSLGTDAPSSTLERAVNYATSRDVLVIAATGNNGSGSVGYPARYANAMAVGATDQNNRRANFSQYGTGIDIVAPGVNVQSTYPGNRYVSMNGTSMATPHVAGAAALVKQRYPSWNATQIRDHLKNTATNLGNSSQFGSGLVNAEAATR

SEQ ID NO: 119 - protein, 269 aa, artificial sequence
  B. gibsonii-clade subtilisin
QQTVPWGITRVQAPAVHNRGITGSGVRVAILDSGISTHEDLNIRGGVSFVPGEPTTADLNGHGTHVAGTVAALNNSIGVIGVAPNAELYAVKVLGANGRGSISGIAQGLEWAAANNMHVANMSLGTDAPSSTLERAVNYATSADVLVIAATGNNGSGTVSYPARYANAMAVGATDQNNRRANFSQYGTGIDIVAPGVNVQSTYPGNRYVSMSGTSMATPHVAGAAALVKQRYPSWNATQIRNHLKNTATNLGNSSQFGSGLVNAEAATR

SEQ ID NO: 120 - protein, 269 aa, artificial sequence
  B. gibsonii-clade subtilisin
QQTVPWGITRVQAPAVHNRGITGSGVRVAILDSGISTHEDLNVRGGVSFVPGEPGTADLNGHGTHVAGTVAALNNSIGVIGVAPNAELYAVKVLGANGRGSISGIAQGLEWAAQNNMHIANMSLGTDAPSSTLERAVNYATSRDVLVIAATGNNGSGSVGYPARYANAMAVGATDQNNRRANFSQYGTGIDIVAPGVNVQSTYPGNRYVSMSGTSMATPHVAGAAALVKQRYPSWNATQIRNHLKNTATNLGNSSQFGSGLVNAEAATR

SEQ ID NO: 121 - protein, 269 aa, artificial sequence
  B. gibsonii-clade subtilisin
QQTVPWGITRVQAPAVHNRGITGSGVRVAILDSGISTHEDLNIRGGASFVPGEPTTADLNGHGTHVAGTVAALDNSIGVVGVAPSADLYAVKVLGANGRGSISGIAQGLEWAAQNNMHIANMSLGTDAPSSTLERAVNYATSADVLVIAATGNNGSGSVGYPARYANAMAVGATDQNNRRANFSQYGTGIDIVAPGVNVQSTYPGNRYVSMNGTSMATPHVAGAAALVKQRYPSWNATQIRNHLKNTATNLGNSSQFGSGLVNAEAATR

SEQ ID NO: 122 - protein, 269 aa, artificial sequence
  B. gibsonii-clade subtilisin
QQTVPWGITRVQAPAVHNRGITGFGVRVAILDSGISTHEDLNIRGGVSFVPGEPTTADLNGHGTHVAGTVAALDNSIGVVGVAPSADLYAVKVLGANGRGSVSGIAQGLEWAAQNNMHIANMSLGTDAPSSTLERAVNYATSRDVLVIAATGNNGSGSVGYPARYANAMAVGATDQNNRRANFSQYGTGIDIVAPGVNVQSTYPGNRYVSMSGTSMATPHVAGAAALVKQRYPSWNATQIRNHLKNTATNLGNSSQFGSGLVNAEAATR

SEQ ID NO: 123 - skipped

SEQ ID NO: 124 - protein, 269 aa, artificial sequence
  B. gibsonii-clade subtilisin
QQTVPWGITRVQAPAVHNRGITGSGVRVAILDSGISTHEDLTIRGGVSFVPGEPTTADLNGHGTHVAGTVAALDNSIGVVGVAPSADLYAVKVLGANGRGSVSGIAQGLEWAAQNNMHIANMSLGSDAPSSTLERAVNYATSRDVLVIAATGNNGSGSVGYPARYANAMAVGATDQNNRRANFSQYGTGIDIVAPGVNVQSTYPGNRYVSMNGTSMATPHVAGAAALVKQRYPSWNATQIRDHLKNTATNLGNSSQFGSGLVNAEAATR

SEQ ID NO: 125 - protein, 269 aa, artificial sequence
  B. gibsonii-clade subtilisin
QQTVPWGITRVQAPAVHNRGITGSGVRVAILDSGISTHEDLTIRGGVSFVPGEPTTADLNGHGTHVAGTVAALNNSIGVVGVAPSADLYAVKVLGANGRGSISGIAQGLEWAAQNNMHIANMSLGSDAPSSTLERAVNYATSRDVLVIAATGNNGSGSVGYPARYANAMAVGATDQNNRRANFSQYGTGIDIVAPGVNVQSTYPGNRYVSMNGTSMATPHVAGAAALVKQRYPSWNATQIRDHLKNTATNLGNSSQFGSGLVNAEAATR

SEQ ID NO: 126 - protein, 269 aa, artificial sequence
  B. gibsonii-clade subtilisin
QQTVPWGITRVQAPAVHNRGITGSGVRVAILDSGISTHEDLTIRGGVSFVPGEPGTADLNGHGTHVAGTVAALNNSIGVVGVAPSADLYAVKVLGANGRGSVSGIAQGLEWAAQNNMHIANMSLGSDAPSSTLERAVNYATSRDVLVIAATGNNGSGSVGYPARYANAMAVGATDQNNRRANFSQYGTGIDIVAPGVNVQSTYPGNRYVSMSGTSMATPHVAGAAALVKQRYPSWNATQIRDHLKNTATNLGNSSQFGSGLVNAEAATR

SEQ ID NO: 127 - protein, 269 aa, artificial sequence
  B. gibsonii-clade subtilisin
QQTVPWGITRVQAPAVHNRGITGSGVKVAILDSGISTHEDLNIRGGVSFVPGEPTTADLNGHGTHVAGTVAALNNSIGVVGVAPSADLYAVKVLGANGRGSVSGIAQGLEWAAQNNMHIANMSLGSDAPSSTLERAVNYATSRDVLVIAATGNNGSGSVGYPARYANAMAVGATDQNNRRANFSQYGTGIDIVAPGVNVQSTYPGNRYVSMSGTSMATPHVAGAAALVKQRYPSWNATQIRDHLKNTATNLGNSSQFGSGLVNAEAATR

SEQ ID NO: 128 - protein, 269 aa, artificial sequence
  B. gibsonii-clade subtilisin
QQTVPWGITRVQAPAVHNRGITGSGVRVAILDSGISTHEDLNIRGGVSFVPGEPTTADLNGHGTHVAGTVAALNNSIGVVGVAPSADLYAVKVLGANGRGSVSGIAQGLEWAAQNNMHIANMSLGSDAPSSTLERAVNYATSADVLVIAATGNNGSGSVGYPARYANAMAVGATDQNNRRANFSQYGTGIDIVAPGVNVQSTYPGNRYVSMNGTSMATPHVAGAAALVKQRYPSWNATQIRDHLKNTATNLGNSSQFGSGLVNAEAATR

SEQ ID NO: 129 - protein, 269 aa, artificial sequence
  B. gibsonii-clade subtilisin
QQTVPWGITRVQAPAVHNRGITGSGVRVAILDSGISTHEDLNIRGGVSFVPGEPTTADLNGHGTHVAGTVAALNNSIGVVGVAPSADLYAVKVLGANGRGSISGIAQGLEWAAQNNMHIANMSLGSDAPSSTLERAVNYATSADVLVIAATGNNGSGSVGYPARYANAMAVGATDQNNRRANFSQYGTGIDIVAPGVNVQSTYPGNRYVSMNGTSMATPHVAGAAALVKQRYPSWNATQIRDHLKNTATNLGNSSQFGSGLVNAEAATR

SEQ ID NO: 130 - protein, 269 aa, artificial sequence
  B. gibsonii-clade subtilisin
QQTVPWGITRVQAPAVHNRGITGSGVRVAILDSGISTHEDLNVRGGVSFVPGEPTTADLNGHGTHVAGTVAALNNSIGVVGVAPSADLYAVKVLGANGRGSVSGIAQGLEWAAQNNMHIANMSLGTDAPSSTLERAVNYATSADVLVIAATGNNGSGSVGYPARYANAMAVGATDQNNRRANFSQYGTGIDIVAPGVNVQSTYPGNRYVSMNGTSMATPHVAGAAALVKQRYPSWNATQIRDHLKNTATNLGNSSQFGSGLVNAEAATR

SEQ ID NO: 131-132 - skipped (2 entries)

SEQ ID NO: 133 - protein, 269 aa, artificial sequence
  B. gibsonii-clade subtilisin
QQTVPWGITRVQAPAVHNRGITGSGVRVAILDSGISTHEDLNVRGGVSFVPGEPTTADLNGHGTHVAGTVAALNNSIGVVGVAPSADLYAVKVLGANGRGSISGIAQGLEWAAQNNMHIANMSLGTDAPSSTLERAVNYATSRDVLVIAATGNNGSGSVGYPARYANAMAVGATDQNNRRANFSQYGTGIDIVAPGVNVQSTYPGNRYVSMNGTSMATPHVAGAAALVKQRYPSWNATQIRDHLKNTATNLGNSSQFGSGLVNAEAATR

SEQ ID NO: 134 - protein, 269 aa, artificial sequence
  B. gibsonii-clade subtilisin
QQTVPWGITRVQAPAVHNRGITGSGVRVAILDSGISTHEDLNVRGGVSFVPGEPGTADLNGHGTHVAGTVAALNNSIGVVGVAPSADLYAVKVLGANGRGSISGIAQGLEWAAQNNMHIANMSLGSDAPSSTLERAVNYATSADVLVIAATGNNGSGSVGYPARYANAMAVGATDQNNRRANFSQYGTGIDIVAPGVNVQSTYPGNRYVSMNGTSMATPHVAGAAALVKQRYPSWNATQIRNHLKNTATNLGNSSQFGSGLVNAEAATR

SEQ ID NO: 135 - protein, 269 aa, artificial sequence
  B. gibsonii-clade subtilisin
QQTVPWGITRVQAPAVHNRGITGSGVRVAILDSGISTHEDLNVRGGVSFVPGEPTTADLNGHGTHVAGTVAALNNSIGVVGVAPSADLYAVKVLGANGRGSISGIAQGLEWAAQNNMHIANMSLGSDAPSSTLERAVNYATSRDVLVIAATGNNGSGSVGYPARYANAMAVGATDQNNRRANFSQYGTGIDIVAPGVNVQSTYPGNRYVSMNGTSMATPHVAGAAALVKQRYPSWNATQIRNHLKNTATNLGNSSQFGSGLVNAEAATR

SEQ ID NO: 136 - protein, 269 aa, artificial sequence
  B. gibsonii-clade subtilisin
QQTVPWGITRVQAPAVHNRGITGSGVRVAILDSGISTHEDLNVRGGVSFVPGEPTTADLNGHGTHVAGTVAALNNSIGVVGVAPSADLYAVKVLGANGRGSVSGIAQGLEWAAQNNMHIANMSLGSDAPSSTLERAVNYATSRDVLVIAATGNNGSGSVGYPARYANAMAVGATDQNNRRANFSQYGTGIDIVAPGVNVQSTYPGNRYVSMSGTSMATPHVAGAAALVKQRYPSWNATQIRDHLKNTATNLGNSSQFGSGLVNAEAATR

SEQ ID NO: 137 - protein, 269 aa, artificial sequence
  B. gibsonii-clade subtilisin
QQTVPWGITRVQAPAVHNRGITGSGVRVAILDSGISTHEDLNVRGGVSFVPGEPTTADLNGHGTHVAGTVAALNNSIGVVGVAPSADLYAVKVLGANGRGSVSGIAQGLEWAAANNMHIANMSLGTDAPSSTLERAVNYATSRDVLVIAATGNNGSGSVGYPARYANAMAVGATDQNNRRANFSQYGTGIDIVAPGVNVQSTYPGNRYVSMNGTSMATPHVAGAAALVKQRYPSWNTTQIRDHLKNTATNLGNSSQFGSGLVNAEAATR

SEQ ID NO: 138 - protein, 269 aa, artificial sequence
  B. gibsonii-clade subtilisin
QQTVPWGITRVQAPAVHNRGITGSGVRVAILDSGISTHEDLNVRGGVSFVPGEPTTADLNGHGTHVAGTVAALNNSIGVVGVAPSADLYAVKVLGANGRGSVSGIAQGLEWAAANNMHIANMSLGSDAPSSTLERAVNYATSRDVLVIAATGNNGSGSVGYPARYANAMAVGATDQNNRRANFSQYGTGIDIVAPGVNVQSTYPGNRYVSMNGTSMATPHVAGAAALVKQRYPSWNATQIRDHLKNTATNLGNSSQFGSGLVNAEAATR

SEQ ID NO: 139 - protein, 269 aa, artificial sequence
  B. gibsonii-clade subtilisin
QQTVPWGITRVQAPAVHNRGITGSGVRVAILDSGISTHEDLNVRGGVSFVPGEPTYADLNGHGTHVAGTVAALNNSIGVVGVAPSADLYAVKVLGANGRGSVSGIAQGLEWAAANNMHIANMSLGSDAPSSTLERAVNYATSRDVLVIAATGNNGSGSVGYPARYANAMAVGATDQNNRRANFSQYGTGIDIVAPGVNVQSTYPGNRYVSMNGTSMATPHVAGAAALVKQRYPSWNATQIRDHLKNTATNLGNSSQFGSGLVNAEAATR

SEQ ID NO: 140 - protein, 269 aa, artificial sequence
  B. gibsonii-clade subtilisin
QQTVPWGITRVQAPAVHNRGITGSGVRVAILDSGIAAHEDLNVRGGVSFVPGEPMTADLNGHGTHVAGTVAALNNSIGVVGVAPSADLYAVKVLGANGRGSVSGIAQGLEWAAANNMHIANMSLGSDAPSSTLERAVNYATSRDVLVIAATGNNGSGSVGYPARYANAMAVGATDQNNRRANFSQYGTGIDIVAPGVNVQSTYPGNRYVSMNGTSMATPHVAGAAALVKQRYPSWNATQIRNHLKNTATNLGNSSQFGSGLVNAEAATR

SEQ ID NO: 141 - protein, 269 aa, artificial sequence
  B. gibsonii-clade subtilisin
QQTVPWGITRVQAPAVHNRGITGSGVRVAILDSGIAAHEDLNVRGGVSFVPGEPTTADLNGHGTHVAGTVAALNNSIGVVGVAPSADLYAVKVLGANGRGSVSGIAQGLEWAAANNMHIASMSLGSDAPSSTLERAVNYATSQDVLVIAATGNNGSGSVGYPARYANAMAVGATDQNNRRANFSQYGTGIDIVAPGVNVQSTYPGNRYVSMNGTSMATPHVAGAAALVKQRYPSWNATQIRNHLKNTATNLGNSSQFGSGLVNAEAATR

SEQ ID NO: 142 - protein, 269 aa, artificial sequence
  B. gibsonii-clade subtilisin
QQTVPWGITRVQAPAVHNRGITGSGVRVAILDSGIAAHEDLNVRGGVSFVPGEPTTADLNGHGTHVAGTVAALNNSIGVVGVAPSADLYAVKVLGANGRGSVSGIAQGLEWAAANNMHIANMSLGSDAPSSTLERAVNYATSRDVLVIAATGNNGSGSVGYPARYANAMAVGATDQNNRRANFSQYGTGIDIVAPGVNVQSTYPGNRYVSMSGTSMATPHVAGAAALVKQRYPSWNATQIRNHLKNTATNLGNSNQFGSGLVNAEAATR

SEQ ID NO: 143 - protein, 269 aa, artificial sequence
  B. gibsonii-clade subtilisin
QQTVPWGITRVQAPAVHNRGITGSGVRVAILDSGISAHEDLNVRGGVSFVPGEPTTADLNGHGTHVAGTVAALNNSIGVVGVAPSADLYAVKVLGANGRGSVSGIAQGLEWAAANNMHIANMSLGSDAPSSTLERAVNYATSRDVLVIAATGNNGSGSVGYPARYANAMAVGATDQNNRRANFSQYGTGIDIVAPGVNVQSTYPGNRYVSMSGTSMATPHVAGAAALVKQRYPSWNATQIRNHLLSTATNLGNSSQFGSGLVNAEAATR

SEQ ID NO: 144 - protein, 269 aa, artificial sequence
  B. gibsonii-clade subtilisin
QQTVPWGITRVQAPAVHNRGITGSGVRVAILDSGISAHEDLNVRGGVSFVPGEPTTADLNGHGTHVAGTVAALNNSIGVVGVAPSADLYAVKVLGANGRGSVSGIAQGLEWAAANNMHIANMSLGSDAPSSTLERAVNYATSQDVLVIAATGNNGSGSVGYPARYANAMAVGATDQNNRRANFSQYGTGIDIVAPGVNVQSTYPGNRYVSMNGTSMATPHVAGAAALVKQRYPSWNATQIRDHLKKTATNLGNSSQFGSGLVNAEAATR

SEQ ID NO: 145 - protein, 269 aa, artificial sequence
  B. gibsonii-clade subtilisin
QQTVPWGITRVQAPAVHNRGITGSGVRVAILDSGISTHEDLNVRGGVSFVPGEPTTADLNGHGTHVAGTVAALDNSIGVIGVAPSADLYAVKVLGANGRGSVSGIAQGLEWAAANNMHIANMSLGTDAPSSTLERAVNYATSRDVLVIAATGNNGSGTVGYPARYANAMAVGATDQNNRRANFSQYGTGIDIVAPGVNVQSTYPGNRYVSMSGTSMATPHVAGAAALVKQRYPSWNATQIRNHLKNTATNLGNSSQFGSGLVNAEAATR

SEQ ID NO: 146 - protein, 269 aa, artificial sequence
  B. gibsonii-clade subtilisin
QQTVPWGITRVQAPAVHNRGITGSGVRVAILDSGISTHEDLNVRGGVSFVPGEPTTADLNGHGTHVAGTVAALDNSIGVIGVAPSADLYAVKVLGANGRGSVSGIAQGLEWAAANNMHIANMSLGSDAPSSTLERAVNYATSRDVLVIAATGNNGSGTVGYPARYANAMAVGATDQNNRRANFSQYGTGIDIVAPGVNVQSTYPGNRYVSMSGTSMATPHVAGAAALVKQRYPSWNATQIRNHLKNTATNLGNSSQFGSGLVNAEAATR

SEQ ID NO: 147 - protein, 269 aa, artificial sequence
  B. gibsonii-clade subtilisin
QQTVPWGITRVQAPAVHNRGITGSGVRVAILDSGISTHEDLNVRGGVSFVPGEPTTADLNGHGTHVAGTVAALDNSIGVIGVAPSADLYAVKVLGANGRGSVSGIAQGLEWAAANNMHIANMSLGTDAPSSTLERAVNYATSRDVLVIAATGNNGSGSVGYPARYANAMAVGATDQNNRRANFSQYGTGIDIVAPGVNVQSTYPGNRYVSMSGTSMATPHVAGAAALVKQRYPSWNATQIRNHLKNTATNLGNSSQFGSGLVNAEAATR

SEQ ID NO: 148 - protein, 269 aa, artificial sequence
  B. gibsonii-clade subtilisin
QQTVPWGITRVQAPAVHNRGITGSGVRVAILDSGISTHEDLNVRGGVSFVPGEPTTADLNGHGTHVAGTVAALDNSIGVVGVAPSADLYAVKVLGANGRGSVSGIAQGLEWAAANNMHIANMSLGSDAPSSTLERAVNYATSRDVLVIAATGNNGSGTVGYPARYANAMAVGATDQNNRRANFSQYGTGIDIVAPGVNVQSTYPGNRYVSMSGTSMATPHVAGAAALVKQRYPSWNATQIRNHLKNTATNLGNSSQFGSGLVNAEAATR

SEQ ID NO: 149 - protein, 269 aa, artificial sequence
  B. gibsonii-clade subtilisin
QQTVPWGITRVQAPAVHNRGITGSGVRVAILDSGISTHEDLNVRGGVSFVPGEPTTADLNGHGTHVAGTVAALDNSIGVVGVAPSADLYAVKVLGANGRGSVSGIAQGLEWAAANNMHIANMSLGSDAPSSTLERAVNYATSRDVLVIAATGNNGSGSVGYPARYANAMAVGATDQNNRRANFSQYGTGIDIVAPGVNVQSTYPGNRYVSMSGTSMATPHVAGAAALVKQRYPSWNATQIRNHLKNTATNLGNSSQFGSGLVNAEAATR

SEQ ID NO: 150 - protein, 269 aa, artificial sequence
  B. gibsonii-clade subtilisin
QQTVPWGITRVQAPAVHNRGITGSGVRVAILDSGISTHEDLNVRGGVSFVPGEPTTADLNGHGTHVAGTVAALDNSIGVIGVAPSADLYAVKVLGANGRGSVSGIAQGLEWAAANNMHIANMSLGSDAPSSTLERAVNYATSRDVLVIAATGNNGSGSVGYPARYANAMAVGATDQNNRRANFSQYGTGIDIVAPGVNVQSTYPGNRYVSMSGTSMATPHVAGAAALVKQRYPSWNATQIRQHLLNTATNLGNSSQFGSGLVNAEAATR

SEQ ID NO: 151 - protein, 269 aa, artificial sequence
  B. gibsonii-clade subtilisin
QQTVPWGITRVQAPAVHNRGITGSGVRVAILDSGISTHEDLNVRGGVSFVPGEPTTADLNGHGTHVAGTVAALDNSIGVVGVAPSADLYAVKVLGANGRGSVSGIAQGLEWAAANNMHIANMSLGSDAPSSTLERAVNYATSRDVLVIAATGNNGSGSVGYPARYANAMAVGATDQNNRRANFSQYGTGIDIVAPGVNVQSTYPGNRYVSMSGTSMATPHVAGAAALVKQRYPSWNATQIRNHLLNTATNLGNSSQFGSGLVNAEAATR

SEQ ID NO: 152 - protein, 269 aa, artificial sequence
  B. gibsonii-clade subtilisin
QQTVPWGITRVQAPAVHNRGITGSGVRVAILDSGISTHEDLNVRGGVSFVPGEPTTADLNGHGTHVAGTVAALDNSIGVVGVAPSADLYAVKVLGANGRGSVSGIAQGLEWAAANNMHIANMSLGSDAPSSTLERAVNYATSRDVLVIAATGNNGSGSVGYPARYANAMAVGATDQNNRRANFSQYGTGIDIVAPGVNVQSTYPGNRYVSMSGTSMATPHVAGAAALVKQRYPSWNATQIRQHLKNTATNLGNSSQFGSGLVNAEAATR

SEQ ID NO: 153 - protein, 269 aa, artificial sequence
  B. gibsonii-clade subtilisin
QQTVPWGITRVQAPAVHNRGITGSGVRVAILDSGISTHEDLTIRGGVSFVPGEPTTADLNGHGTHVAGTVAALNNSIGVVGVAPSADLYAVKVLGANGRGSVSGIAQGLEWAAANNMHIANMSLGSDAPSSTLERAVNYATSRDVLVIAATGNNGSGTVGYPARYANAMAVGATDQNNRRANFSQYGTGIDIVAPGVNVQSTYPGNRYVSMSGTSMATPHVAGAAALVKQRYPSWNATQIRNHLKNTATNLGNSSQFGSGLVNAEAATR

SEQ ID NO: 154 - protein, 269 aa, artificial sequence
  B. gibsonii-clade subtilisin
QQTVPWGITRVQAPAVHNRGITGSGVRVAILDSGISTHEDLNVRGGVSFVPGEPTTADLNGHGTHVAGTVAALNNSIGVVGVAPSADLYAVKVLGANGRGSISGIAQGLEWAAANNMHIANMSLGSDAPSSTLERAVNYATSRDVLVIAATGNNGSGSVGYPARYANAMAVGATDQNNRRANFSQYGTGIDIVAPGVNVQSTYPGNRYVSMSGTSMATPHVAGAAALVKQRYPSWNATQIRNHLKNTATNLGNSSQFGSGLVNAEAATR

SEQ ID NO: 155 - protein, 269 aa, artificial sequence
  B. gibsonii-clade subtilisin
QQTVPWGITRVQAPAVHNRGITGSGVRVAILDSGISTHEDLNVRGGVSFVPGEPTTADLNGHGTHVAGTVAALNNSIGVVGVAPSADLYAVKVLGANGRGSVSGIAQGLEWAAANNMHIANMSLGTDAPSSTLERAVNYATSRDVLVIAATGNNGSGSVGYPARYANAMAVGATDQNNRRANFSQYGTGIDIVAPGVNVQSTYPGNRYVSMSGTSMATPHVAGAAALVKQRYPSWNATQIRNHLKNTATNLGNSSQFGSGLVNAEAATR

SEQ ID NO: 156 - protein, 269 aa, artificial sequence
  B. gibsonii-clade subtilisin
QQTVPWGISRVQAPAVHNRGITGSGVRVAILDSGISTHEDLNVRGGVSFVPGEPTTADLNGHGTHVAGTVAALNNSIGVVGVAPSADLYAVKVLGANGRGSVSGIAQGLEWAAANNMHIANMSLGSDAPSSTLERAVNYATSRDVLVIAATGNNGSGSVGYPARYANAMAVGATDQNNRRANFSQYGTGIDIVAPGINVQSTYPGNRYVSMNGTSMATPHVAGAAALVKQRYPSWNATQIRNHLKNTATNLGNSSQFGSGLVNAEAATR

SEQ ID NO: 157 - protein, 269 aa, artificial sequence
  B. gibsonii-clade subtilisin
QQTVPWGITRVQAPAVHNRGITGSGVRVAILDSGISTHEDLNVRGGVSFVPGEPTTADLNGHGTHVAGTVAALNNSIGVVGVAPSADLYAVKVLGANGRGSVSGIAQGLEWAAANNMHIANMSLGSDAPSSTLERAVNYATSRDVLVIAATGNNGSGSVGYPARYANAMAVGATDQNNRRANFSQYGTGLDIVAPGVNVQSTYPGNRYVSMNGTSMATPHVAGVAALVKQRYPSWNATQIRNHLKNTATNLGNSSQFGSGLVNAEAATR

SEQ ID NO: 158 - protein, 269 aa, artificial sequence
  B. gibsonii-clade subtilisin
QQTIPWGITRVQAPAVHNRGITGSGVRVAILDSGISTHEDLNVRGGVSFVPGEPTTADLNGHGTHVAGTVAALNNSIGVVGVAPSADLYAVKVLGANGRGSVSGIAQGLEWAAANNMHIANMSLGSDAPSSTLERAVNYATSRDVLVIAATGNNGSGSVGYPARYANAMAVGATDQNNRRASFSQYGTGIDIVAPGVNVQSTYPGNRYVSMNGTSMATPHVAGAAALVKQRYPSWNATQIRNHLKNTATNLGNSSQFGSGLVNAEAATR

SEQ ID NO: 159 - protein, 275 aa, artificial sequence
  Consensus sequence of Figure 7
  MISC_FEATURE (38)..(38): Xaa can be any amino acid
  MISC_FEATURE (57)..(57): Xaa can be any amino acid
  MISC_FEATURE (116)..(116): Xaa can be any amino acid
  MISC_FEATURE (159)..(162): Xaa can be any amino acid
QQTVPWGITRVQAPAVHNRGITGSGVRVAILDSGISTXHEDLNVRGGVSFVPGEPTXTADLNGHGTHVAGTVAALNNSIGVVGVAPSADLYAVKVLGANGRGSVSGIAQGLEWAAXNNMHIANMSLGSDAPSSTLERAVNYATSRDVLVIAATGNNGSXXXXGSVGYPARYANAMAVGATDQNNRRANFSQYGTGIDIVAPGVNVQSTYPGNRYVSMNGTSMATPHVAGAAALVKQRYPSWNATQIRNHLKNTATNLGNSSQFGSGLVNAEAATR

SEQ ID NO: 160 - protein, 269 aa, artificial sequence
  B. gibsonii-clade subtilisin
QQTVPWGITRVQAPAVHNRGITGSGVRVAILDSGISTHEDLNVRGGVSFVPGEPTTADLNGHGTHVAGTVAALDNSIGVVGVAPSADLYAVKVLGANGRGSVSGIAQGLEWAAANNMHIANMSLGTDAPSSTLERAVNYATSRDVLVIAATGNNGSGTVGYPARYANAMAVGATDQNNRRANFSQYGTGIDIVAPGVNVQSTYPGNRYVSMSGTSMATPHVAGAAALVKQRYPSWNATQIRQHLKNTATNLGNSSQFGSGLVNAEAATR

SEQ ID NO: 161 - protein, 269 aa, artificial sequence
  B. gibsonii-clade subtilisin
QQTVPWGITRVQAPAVHNRGITGSGVRVAILDSGISTHEDLNVRGGVSFVPGEPTTADLNGHGTHVAGTVAALDNSIGVIGVAPSADLYAVKVLGANGRGSVSGIAQGLEWAAANNMHIANMSLGTDAPSSTLERAVNYATSRDVLVIAATGNNGSGTVGYPARYANAMAVGATDQNNRRANFSQYGTGIDIVAPGVNVQSTYPGNRYVSMSGTSMATPHVAGAAALVKQRYPSWNATQIRQHLKNTATNLGNSSQFGSGLVNAEAATR

SEQ ID NO: 162 - protein, 269 aa, artificial sequence
  B. gibsonii-clade subtilisin
QQTVPWGITRVQAPAVHNRGITGSGVRVAILDSGISTHEDLNVRGGVSFVPGEPTTADLNGHGTHVAGTVAALDNSIGVVGVAPSADLYAVKVLGANGRGSVSGIAQGLEWAAANNMHIANMSLGTDAPSSTLERAVNYATSRDVLVIAATGNNGSGTVGYPARYANAMAVGATDQNNRRANFSQYGTGIDIVAPGVNVQSTYPGNRYVSMSGTSMATPHVAGAAALVKQRYPSWNATQIRQHLLNTATNLGNSSQFGSGLVNAEAATR

SEQ ID NO: 163 - protein, 269 aa, artificial sequence; identical to SEQ ID NO: 148
  B. gibsonii-clade subtilisin

SEQ ID NO: 164 - protein, 269 aa, artificial sequence
  B. gibsonii-clade subtilisin
QQTVPWGITRVQAPAVHNRGITGSGVRVAILDSGISTHEDLNVRGGVSFVPGEPTTADLNGHGTHVAGTVAALDNSIGVIGVAPSADLYAVKVLGANGRGSVSGIAQGLEWAAANNMHIANMSLGTDAPSSTLERAVNYATSRDVLVIAATGNNGSGTVGYPARYANAMAVGATDQNNRRANFSQYGTGIDIVAPGVNVQSTYPGNRYVSMSGTSMATPHVAGAAALVKQRYPSWNATQIRQHLLNTATNLGNSSQFGSGLVNAEAATR

SEQ ID NO: 165 - protein, 269 aa, artificial sequence
  B. gibsonii-clade subtilisin
QQTVPWGITRVQAPAVHNRGITGSGVRVAILDSGISTHEDLNVRGGVSFVPGEPTTADLNGHGTHVAGTVAALDNSIGVIGVAPSADLYAVKVLGANGRGSVSGIAQGLEWAAANNMHIANMSLGTDAPSSTLERAVNYATSRDVLVIAATGNNGSGTVGYPARYANAMAVGATDQNNRRANFSQYGTGIDIVAPGVNVQSTYPGNRYVSMSGTSMATPHVAGAAALVKQRYPSWNATQIRNHLLNTATNLGNSSQFGSGLVNAEAATR

SEQ ID NO: 166 - protein, 269 aa, artificial sequence
  B. gibsonii-clade subtilisin
QQTVPWGITRVQAPAVHNRGITGSGVRVAILDSGISTHEDLNIRGGVSFVPGEPTYADLNGHGTHVAGTVAALNNSIGVVGVAPSADLYAVKVLGANGRGSVSGIAQGLEWAAQNNMHIANMSLGSDFPSSTLERAVNYATSADVLVIAATGNNGSGSVGYPARYANAMAVGATDQNNRRANFSQYGTGIDIVAPGVNVQSTYPGNRYVSMNGTSMATPHVAGAAALVKQRYPSWNATQIRDHLKNTATNLGNSSQFGSGLVNAEAATR

SEQ ID NO: 167 - protein, 269 aa, artificial sequence
  B. gibsonii-clade subtilisin
QQTVPWGITRVQAPAVHNRGITGSGVRVAILDSGISTHEDLTVSGGVSFVPGEPTTADLNGHGTHVAGTVAALDNSIGVVGVAPSADLYAVKVLGANGRGSISGIAQGLEWAATNNMHIANMSLGTDAPSSTLERAVNYATSRDVLVIAATGNNGSGTVSYPARYANAMAVGATDQNNRRANFSQYGTGIDIVAPGVNVQSTYPGNRYVSMNGTSMATPHVAGAAALVKQRYPSWNATQIRDHLKNTATNLGNSSQFGSGLVNAEAATR

SEQ ID NO: 168 - protein, 269 aa, artificial sequence
  B. gibsonii-clade subtilisin
QQTVPWGITRVQAPAVHNRGITGSGVRVAILDSGISTHEDLNVRGGVSFVPGEPGTADLNGHGTHVAGTVAALDNSIGVVGVAPSADLYAVKVLGANGRGSISGIAQGLEWAAQNNMHIANMSLGTDAPSSTLERAVNYATSRDVLVIAATGNNGSGTVGYPARYANAMAVGATDQNNRRANFSQYGTGIDIVAPGVNVQSTYPGNRYVSMNGTSMATPHVAGAAALVKQRYPSWNATQIRDHLKNTATNLGNSSQFGSGLVNAEAATR

SEQ ID NO: 169 - protein, 269 aa, artificial sequence
  B. gibsonii-clade subtilisin
QQTVPWGITRVQAPAVHNRGITGSGVRVAILDSGISTHEDLNVRGGVSFVPGEPGTADLNGHGTHVAGTVAALDNSIGVVGVAPSADLYAVKVLGANGRGSVSGIAQGLEWAAQNNMHIANMSLGTDAPSSTLERAVNYATSADVLVIAATGNNGSGTVGYPARYANAMAVGATDQNNRRANFSQYGTGIDIVAPGVNVQSTYPGNRYVSMSGTSMATPHVAGAAALVKQRYPSWNATQIRNHLKNTATNLGNSSQFGSGLVNAEAATR

SEQ ID NO: 170 - protein, 269 aa, artificial sequence
  B. gibsonii-clade subtilisin
QQTVPWGITRVQAPAVHNRGITGSGVRVAILDSGISTHEDLNVRGGVSFVPGEPGTADLNGHGTHVAGTVAALDNSIGVVGVAPSADLYAVKVLGANGRGSVSGIAQGLEWAAQNNMHIANMSLGTDAPSSTLERAVNYATSRDVLVIAATGNNGSGSVGYPARYANAMAVGATDQNNRRANFSQYGTGIDIVAPGVNVQSTYPGNRYVSMNGTSMATPHVAGAAALVKQRYPSWNATQIRDHLKNTATNLGNSSQFGSGLVNAEAATR

SEQ ID NO: 171 - protein, 269 aa, artificial sequence
  B. gibsonii-clade subtilisin
QQTVPWGITRVQAPAVHNRGITGSGVRVAILDSGISTHEDLNVRGGVSFVPGEPGTADLNGHGTHVAGTVAALNNSIGVVGVAPSADLYAVKVLGANGRGSISGIAQGLEWAAQNNMHIANMSLGTDAPSSTLERAVNYATSADVLVIAATGNNGSGSVGYPARYANAMAVGATDQNNRRANFSQYGTGIDIVAPGVNVQSTYPGNRYVSMNGTSMATPHVAGAAALVKQRYPSWNATQIRNHLKNTATNLGNSSQFGSGLVNAEAATR

SEQ ID NO: 172 - protein, 269 aa, artificial sequence
  B. gibsonii-clade subtilisin
QQTVPWGITRVQAPAVHNRGITGSGVRVAILDSGISTHEDLNVRGGVSFVPGEPTTADLNGHGTHVAGTVAALNNSIGVVGVAPSADLYAVKVLGANGRGSISGIAQGLEWAAQNNMHIANMSLGTDAPSSTLERAVNYATSADVLVIAATGNNGSGSVGYPARYANAMAVGATDQNNRRANFSQYGTGIDIVAPGVNVQSTYPGNRYVSMNGTSMATPHVAGAAALVKQRYPSWNATQIRDHLKNTATNLGNSSQFGSGLVNAEAATR

SEQ ID NO: 173 - protein, 269 aa, artificial sequence; identical to SEQ ID NO: 138
  B. gibsonii-clade subtilisin

SEQ ID NO: 174 - protein, 269 aa, artificial sequence
  B. gibsonii-clade subtilisin
QQTVPWGITRVQAPAVHNRGITGSGVRVAILDSGISTHEDLNVRGGVSFVPGEPTTADLNGHGTHVAGTVAALNNSIGVVGVAPSADLYAVKVLGANGRGSVSGIAQGLEWAAANNMHIANMSLGTDAPSSTLERAVNYATSADVLVIAATGNNGSGTVGYPARYANAMAVGATDQNNRRANFSQYGTGIDIVAPGVNVQSTYPGNRYVSMNGTSMATPHVAGAAALVKQRYPSWNATQIRDHLKNTATNLGNSSQFGSGLVNAEAATR

SEQ ID NO: 175 - protein, 269 aa, artificial sequence
  B. gibsonii-clade subtilisin
QQTVPWGITRVQAPAVHNRGITGSGVRVAILDSGISTHEDLNVRGGVSFVPGEPTTADLNGHGTHVAGTVAALNNSIGVVGVAPSADLYAVKVLGANGRGSVSGIAQGLEWAAPNNMHIANMSLGTDAPSSTLERAVNYATSTDVLVIAATGNNGSGTVGYPARYANAMAVGATDQNNRRANFSQYGTGIDIVAPGVNVQSTYPGNRYVSMKGTSMATPHVAGAAALVKQRYPSWNATQIRDHLKNTATNLGNSSQFGSGLVNAEAATR

SEQ ID NO: 176 - protein, 269 aa, artificial sequence
  B. gibsonii-clade subtilisin
QQTVPWGITRVQAPAVHNRGITGSGVRVAILDSGISTHEDLTIRGGVSFVPGEPTTADLNGHGTHVAGTVAALDNSIGVVGVAPSADLYAVKVLGANGRGSISGIAQGLEWAAQNNMHIANMSLGTDAPSSTLERAVNYATSRDVLVIAATGNNGSGSVGYPARYANAMAVGATDQNNRRANFSQYGTGIDIVAPGVNVQSTYPGNRYVSMNGTSMATPHVAGAAALVKQRYPSWNATQIRDHLKNTATNLGNSSQFGSGLVNAEAATR

SEQ ID NO: 177 - protein, 269 aa, artificial sequence
  B. gibsonii-clade subtilisin
QQTVPWGITRVQAPAVHNRGITGSGVRVAILDSGISTHEDLNVRGGVSFVPGEPTYADLNGHGTHVAGTVAALDNSIGVVGVAPSADLYAVKVLGANGRGSVSGIAQGLEWAAQNNMHIANMSLGTDAPSSTLERAVNYATSADVLVIAATGNNGSGSVGYPARYANAMAVGATDQNNRRANFSQYGTGIDIVAPGVNVQSTYPGNRYVSMNGTSMATPHVAGAAALVKQRYPSWNATQIRDHLKNTATNLGNSSQFGSGLVNAEAATR

SEQ ID NO: 178 - protein, 269 aa, artificial sequence
  B. gibsonii-clade subtilisin
QQTVPWGITRVQAPAVHNRGITGSGVRVAILDSGISTHEDLNVRGGVSFVPGEPTYADLNGHGTHVAGTVAALNNSIGVVGVAPSADLYAVKVLGANGRGSVSGIAQGLEWAAQNNMHVANMSLGTDAPSSTLERAVNYATSRDVLVIAATGNNGSGSVGYPARYANAMAVGATDQNNRRANFSQYGTGIDIVAPGVNVQSTYPGNRYVSMNGTSMATPHVAGAAALVKQRYPSWNATQIRNHLKNTATNLGNSSQYGSGLVNAEAATR

SEQ ID NO: 179 - protein, 269 aa, artificial sequence
  B. gibsonii-clade subtilisin
QQTVPWGITRVQAPAVHNRGITGSGVRVAILDSGISTHEDLNVRGGVSFVPGEPGYADLNGHGTHVAGTVAALDNSIGVVGVAPSADLYAVKVLGANGRGSISGIAQGLEWAAQNNMHIANMSLGTDAPSSTLERAVNYATSRDVLVIAATGNNGSGSVGYPARYANAMAVGATDQNNRRANFSQYGTGIDIVAPGVNVQSTYPGNRYVSMNGTSMATPHVAGAAALVKQRYPSWNATQIRNHLKNTATNLGNSSQFGSGLVNAEAATR

SEQ ID NO: 180 - protein, 269 aa, artificial sequence
  B. gibsonii-clade subtilisin
QQTVPWGITRVQAPAVHNRGITGSGVRVAILDSGISTHEDLNVRGGVSFVPGEPTTADLNGHGTHVAGTVAALNNSIGVVGVAPSADLYAVKVLGANGRGSVSGIAQGLEWAAANNMHVANMSLGTDAPSSTLERAVNYATSRDVLVIAATGNNGSGTVSYPARYANAMAVGATDQNNRRANFSQYGTGIDIVAPGVNVQSTYPGNRYVSMNGTSMATPHVAGAAALVKQRYPSWNATQIRDHLKNTATNLGNSSQYGSGLVNAEAATR

SEQ ID NO: 181 - protein, 269 aa, artificial sequence
  B. gibsonii-clade subtilisin
QQTVPWGITRVQAPAVHNRGITGSGVKVAILDSGISTHEDLNVRGGVSFVPGEPTYADLNGHGTHVAGTVAALNNSIGVVGVAPSADLYAVKVLGANGRGSISGIAQGLEWAAQNNMHIANMSLGTDAPSSTLERAVNYATSRDVLVIAATGNNGSGSVGYPARYANAMAVGATDQNNRRANFSQYGAGLDIVAPGVNVQSTYPGNRYVSMNGTSMATPHVAGAAALVKQRYPSWNATQIRNHLKNTATNLGNSSQYGSGLVNAEAATR

SEQ ID NO: 182 - protein, 269 aa, artificial sequence
  B. gibsonii-clade subtilisin
QQTVPWGITRVQAPAVHNRGITGSGVKVAILDSGISTHEDLNVRGGVSFVPGEPTNADLNGHGTHVAGTVAALNNSIGVVGVAPSADLYAVKVLGANGRGSVSGIAQGLEWAAPNNMHIANMSLGTDAPSSTLERAVNYATSTDVLVIAATGNNGSGSIGYPARYANAMAVGATDQNNRRANFSQYGTGIDIVAPGVNVQSTYPGNRYVSMTGTSMATPHVAGAAALVKQRYPSWNATQIRNHLKNTATNLGNSSQYGSGLVNAEAATR

SEQ ID NO: 183 - protein, 269 aa, artificial sequence
  B. gibsonii-clade subtilisin
QQTVPWGITRVQAPAVHNRGITGSGVRVAILDSGISTHEDLNVRGGVSFVPGEPTTADLNGHGTHVAGTVAALNNSIGVVGVAPSADLYAVKVLGANGRGSISGIAQGLEWAAANNMHVANMSLGTDAPSSTLERAVNYATSRDVLVIAATGNNGSGSVGYPARYANAMAVGATDQNNRRANFSQYGTGIDIVAPGVNVQSTYPGNRYVSMNGTSMATPHVAGAAALVKQRYPSWNATQIRNHLKNTATNLGNSSQYGSGLVNAEAATR

SEQ ID NO: 184 - protein, 269 aa, artificial sequence
  B. gibsonii-clade subtilisin
QQTVPWGITRVQAPAVHNRGITGSGVRVAILDSGISTHEDLNVRGGVSFVPGEPTYADLNGHGTHVAGTVAALNNSIGVVGVAPSADLYAVKVLGANGRGSVSGIAQGLEWAAQNNMHVANMSLGTDAPSSTLERAVNYATSRDVLVIAATGNNGSGTISYPARYANAMAVGATDQNNRRANFSQYGTGIDIVAPGVNVQSTYPGNRYVSMNGTSMATPHVAGAAALVKQRYPSWNATQIRNHLKNTATNLGNSSQYGSGLVNAEAATR

SEQ ID NO: 185 - protein, 269 aa, artificial sequence
  B. gibsonii-clade subtilisin
QQTVPWGITRVQAPAVHNRGITGSGVKVAILDSGISTHEDLNIRGGVSFVPGEPTTADLNGHGTHVAGTVAALNNSIGVVGVAPSADLYAVKVLGANGRGSVSGIAQGLEWAAQNNMHVANMSLGTDAPSSTLERAVNYATSRDVLVIAATGNNGSGSVSYPARYANAMAVGATDQNNRRANFSQYGTGIDIVAPGVNVQSTYPGNRYVSMNGTSMATPHVAGAAALVKQRYPSWNATQIRDHLKNTATNLGNSSQYGSGLVNAEAATR

SEQ ID NO: 186 - protein, 269 aa, artificial sequence
  B. gibsonii-clade subtilisin
QQTVPWGITRVQAPAVHNRGITGSGVRVAILDSGISTHEDLNVRGGVSFVPGEPTTADLNGHGTHVAGTVAALDNSIGVVGVAPSADLYAVKVLGANGRGSVSGIAQGLEWAAANNMHIANMSLGTDAPSSTLERAVNYATSRDVLVIAATGNNGSGSVGYPARYANAMAVGATDQNNRRANFSQYGAGLDIVAPGVNVQSTYPGNRYVSMNGTSMATPHVAGAAALVKQRYPSWNATQIRNHLKNTATNLGNSSQYGSGLVNAEAATR

SEQ ID NO: 187 - protein, 269 aa, artificial sequence
  B. gibsonii-clade subtilisin
QQTVPWGITRVQAPAVHNRGITGSGVRVAILDSGIANHEDLNVRGGVSFVPGEPTTADLNGHGTHVAGTVAALNNSIGVVGVAPSADLYAVKVLGANGRGSVSGIAQGLEWAAANNMHIANMSLGSDAPSSTLERAVNYATSRDVLVIAATGNNGSGSVGYPARYANAMAVGATDQNNRRANFSQYGTGIDIVAPGVNVQSTYPGNRYVSMNGTSMATPHVAGAAALVKQRYPSWNATQIRDHLLSTATNLGNSNQFGSGLVNAEAATR

SEQ ID NO: 188 - protein, 269 aa, artificial sequence
  B. gibsonii-clade subtilisin
QQTVPWGITRVQAPAVHNRGITGSGVRVAILDSGIAAHEDLNVRGGVSFVPGEPTTADLNGHGTHVAGTVAALDNSIGVVGVAPSADLYAVKVLGANGRGSVSGIAQGLEWAAANNMHIANMSLGSDAPSSTLERAVNYATSRDVLVIAATGNNGSGSVGYPARYANAMAVGATDQNNRRANFSQYGTGIDIVAPGVNVQSTYPGNRYVSMNGTSMATPHVAGVAALVKQRYPSWNATQIRNHLKNTATNLGNSNQFGSGLVNAEAATR

SEQ ID NO: 189 - protein, 269 aa, artificial sequence
  B. gibsonii-clade subtilisin
QQTVPWGISRVQAPAVHNRGITGSGVRVAILDSGIAAHEDLNVRGGVSFVPGEPTTADLNGHGTHVAGTVAALNNSIGVVGVAPSADLYAVKVLGANGRGSVSGIAQGLEWAAANNMHIANMSLGSDAPSSTLERAVNYATSQDVLVIAATGNNGSGSVGYPARYANAMAVGATDQNNRRASFSQYGAGLDIVAPGVNVQSTYPGNRYVSMNGTSMATPHVAGAAALVKQRYPSWNATQIRNHLKNTATNLGNSSQFGSGLVNAEAATR

SEQ ID NO: 190 - protein, 269 aa, artificial sequence
  B. gibsonii-clade subtilisin
QQTVPWGITRVQAPAVHNRGITGSGVRVAILDSGISTHEDLNVRGGVSFVPGESTYQDLNGHGTHVAGTVAALDNSIGVVGVAPSADLYAVKVLGANGRGSVSGIAQGLEWAAANNMHIASMSLGSDAPSSTLERAVNYATSRDVLVIAATGNNGSGTVGYPARYANAMAVGATDQNNRRANFSQYGTGIDIVAPGVNVQSTYPGNRYVSMNGTSMATPHVAGVAALVKQRYPSWNATQIRNHLKNTATNLGNSNQFGSGLVNAEAATR

SEQ ID NO: 191 - protein, 269 aa, artificial sequence
  B. gibsonii-clade subtilisin
QQTVPWGITRVQAPAVHNRGITGSGVRVAILDSGISTHEDLNVRGGVSFVPGEPTTADLNGHGTHVAGTVAALNNSIGVVGVAPSADLYAVKVLGANGRGSVSGIAQGLEWAAANNMHIANMSLGSDAPSSTLERAVNYATSQDVLVIAATGNNGSGSVGYPARYANAMAVGATDQNNRRANFSQYGTGIDIVAPGVNVQSTYPGNRYVSMSGTSMATPHVAGVAALVKQRNPSWNATQIRNHLLSTATNLGNSNQFGSGLVNAEAATR

SEQ ID NO: 192 - protein, 269 aa, artificial sequence
  B. gibsonii-clade subtilisin
QQTVPWGITRVQAPAVHNRGITGSGVRVAILDSGISAHEDLNVRGGVSFVPGEPTTADLNGHGTHVAGTVAALNNSIGVVGVAPSADLYAVKVLGANGRGSVSGIAQGLEWAAANNMHIANMSLGSDAPSSTLERAVNYATSRDVLVIAATGNNGSGSVGYPARYANAMAVGATDQNNRRANFSQYGTGIDIVAPGVNVQSTYPGNRYVSMNGTSMATPHVAGVAALVKQRYPSWNATQIRDHLKSTATNLGNSNQFGSGLVNAEAATR

SEQ ID NO: 193 - protein, 269 aa, artificial sequence
  B. gibsonii-clade subtilisin
QQTVPWGITRVQAPAVHNRGITGSGVRVAILDSGISTHEDLNVRGGVSFVPGEPTTADLNGHGTHVAGTVAALNNSIGVVGVAPSADLYAVKVLGANGRGSVSGIAQGLEWAAANNMHIASMSLGSDAPSSTLERAVNYATSRDVLVIAATGNNGSGSVGYPARYANAMAVGATDQNNRRASFSQYGTGLDIVAPGVNVQSTYPGNRYVSMNGTSMATPHVAGAAALVKQRYPSWNATQIRNHLLSTATNLGNSNQFGSGLVNAEAATR

SEQ ID NO: 194 - protein, 269 aa, artificial sequence
  B. gibsonii-clade subtilisin
QQTIPWGISRVQAPAVHNRGITGSGVRVAILDSGISTHEDLNVRGGVSFVPGEPTTADLNGHGTHVAGTVAALNNSIGVVGVAPSADLYAVKVLGANGRGSVSGIAQGLEWAAANNMHIASMSLGSDAPSSTLERAVNYATSQDVLVIAATGNNGSGSVGYPARYANAMAVGATDQNNRRANFSQYGTGIDIVAPGVNVQSTYPGNRYVSMNGTSMATPHVAGIAALVKQKYPSWNATQIRNHLLNTATNLGNSSQFGSGLVNAEAATR

SEQ ID NO: 195 - protein, 269 aa, artificial sequence
  B. gibsonii-clade subtilisin
QQTVPWGITRVQAPAVHNRGITGSGVRVAILDSGISTHEDLNVRGGVSFVPGEPTTADLNGHGTHVAGTVAALDNSIGVVGVAPSADLYAVKVLGANGRGSISGIAQGLEWAAANNMHIASMSLGSDAPSSTLERAVNYATSQDVLVIAATGNNGSGSVGYPARYANAMAVGATDQNNRRANFSQYGTGIDIVAPGVNVQSTYPGNRYVSMNGTSMATPHVAGAAALVKQRYPSWNATQIRNHLKNTATNLGNSSQFGSGLVNAEAATR

SEQ ID NO: 196 - protein, 269 aa, artificial sequence
  B. gibsonii-clade subtilisin
QQTVPWGITRVQAPAVHNRGITGSGVRVAILDSGISTHEDLNVRGGVSFVPGEPTTADLNGHGTHVAGTVAALNNSIGVVGVAPSADLYAVKVLGANGRGSVSGIAQGLEWAAANNMHIASMSLGSDAPSSTLERAVNYATSRDVLVIAATGNNGSGSVGYPARYANAMAVGATDQNNRRANFSQYGTGIDIVAPGVNVQSTYPGNRYVSMNGTSMATPHVAGAAALVKQRYPSWNATQIRNHLKSTATNLGNSNQFGSGLVNAEAATR

SEQ ID NO: 197 - protein, 269 aa, artificial sequence
  B. gibsonii-clade subtilisin
QQTVPWGITRVQAPAVHNRGITGSGVRVAILDSGISTHEDLNVRGGVSFVPGEPTTADLNGHGTHVAGTVAALDNSIGVVGVAPSADLYAVKVLGANGRGSVSGIAQGLEWAAQNNMHVANMSLGTDAPSSTLERAVNYATSRDVLVIAATGNNGSGSVGYPARYANAMAVGATDQNNRRANFSQYGTGIDIVAPGVNVQSTYPGNRYVSMNGTSMATPHVAGAAALVKQRYPSWNATQIRNHLKNTATNLGNSSQFGSGLVNAEAATR

SEQ ID NO: 198 - protein, 275 aa, artificial sequence
  Consensus sequence Figure 8
  MISC_FEATURE (37)..(37): Xaa can be any amino acid
  MISC_FEATURE (57)..(57): Xaa can be any amino acid
  MISC_FEATURE (116)..(116): Xaa can be any amino acid
  MISC_FEATURE (161)..(164): Xaa can be any amino acid
  MISC_FEATURE (248)..(248): Xaa can be any amino acid
QQTVPWGITRVQAPAVHNRGITGSGVRVAILDSGISXTHEDLNVRGGVSFVPGEPTXTADLNGHGTHVAGTVAALNNSIGVVGVAPSADLYAVKVLGANGRGSVSGIAQGLEWAAXNNMHIANMSLGTDAPSSTLERAVNYATSRDVLVIAATGNNGSGSXXXXVGYPARYANAMAVGATDQNNRRANFSQYGTGIDIVAPGVNVQSTYPGNRYVSMNGTSMATPHVAGAAALVKQRYPSWNATQIRXHLKNTATNLGNSSQFGSGLVNAEAATR

SEQ ID NO: 199 - protein, 269 aa, artificial sequence
  Consensus sequence Figure 12
  MISC_FEATURE (143)..(143): Xaa can be any amino acid
QQTVPWGITRVQAPAVHNRGITGSGVRVAILDSGISAHSDLNIRGGASFVPGEPTTADLNGHGTHVAGTVAALDNSIGVVGVAPSADLYAVKVLGANGRGSISGIAQGLEWAATNNMHIANMSLGTDAPSSTLERAVNYATSXDVLVIAATGNNGSGSVGYPARYANAMAVGATDQNNRRANFSQYGTGIDIVAPGVNVQSTYPGNRYVSMNGTSMATPHVAGAAALVKQRYPSWNATQIRDHLKNTATNLGNSSQFGSGLVNAEAATR

SEQ ID NO: 200 - protein, 269 aa, artificial sequence
  B. gibsonii-clade subtilisin
QQTVPWGITRVQAPAVHNRGITGSGVRVAILDSGISTHSDLNIRGGASFVPGEPTTADLNGHGTHVAGTVAALNNSIGVIGVAPNAELYAVKVLGANGSGSVSGIAQGLEWAATNNMHIANMSLGSDFPSSTLERAVNYATSRDVLVIAATGNNGSGSVGYPARYANAMAVGATDQNNRRANFSQYGTGIDIVAPGVNVQSTYPGNRYVSMNGTSMATPHVAGAAALVKQRYPSWNATQIRNHLKNTATNLGNSSQFGSGLVNAEAATR

SEQ ID NO: 201 - protein, 269 aa, artificial sequence
  B. gibsonii-clade subtilisin
QQTVPWGITRVQAPAVHNRGITGSGVRVAILDSGISAHEDLNIRGGASFVPGEPTTADLNGHGTHVAGTVAALNNSIGVIGVAPNAELYAVKVLGANGSGSVSGIAQGLEWAATNNMHIANMSLGSDFPSSTLERAVNYATSRDVLVIAATGNNGSGSVGYPARYANAMAVGATDQNNRRANFSQYGTGIDIVAPGVNVQSTYPGNRYVSMNGTSMATPHVAGAAALVKQRYPSWNATQIRNHLKNTATNLGNSSQFGSGLVNAEAATR

SEQ ID NO: 202 - protein, 269 aa, artificial sequence
  B. gibsonii-clade subtilisin
QQTVPWGITRVQAPAVHNRGITGSGVRVAILDSGISAHSDLNIRGGVSFVPGEPTTADLNGHGTHVAGTVAALNNSIGVIGVAPNAELYAVKVLGANGSGSVSGIAQGLEWAATNNMHIANMSLGSDFPSSTLERAVNYATSRDVLVIAATGNNGSGSVGYPARYANAMAVGATDQNNRRANFSQYGTGIDIVAPGVNVQSTYPGNRYVSMNGTSMATPHVAGAAALVKQRYPSWNATQIRNHLKNTATNLGNSSQFGSGLVNAEAATR

SEQ ID NO: 203 - protein, 269 aa, artificial sequence
  B. gibsonii-clade subtilisin
QQTVPWGITRVQAPAVHNRGITGSGVRVAILDSGISAHSDLNIRGGASFVPGEPTYADLNGHGTHVAGTVAALNNSIGVIGVAPNAELYAVKVLGANGSGSVSGIAQGLEWAATNNMHIANMSLGSDFPSSTLERAVNYATSRDVLVIAATGNNGSGSVGYPARYANAMAVGATDQNNRRANFSQYGTGIDIVAPGVNVQSTYPGNRYVSMNGTSMATPHVAGAAALVKQRYPSWNATQIRNHLKNTATNLGNSSQFGSGLVNAEAATR

SEQ ID NO: 204 - protein, 269 aa, artificial sequence; identical to SEQ ID NO: 87
  B. gibsonii-clade subtilisin

SEQ ID NO: 205 - protein, 269 aa, artificial sequence
  B. gibsonii-clade subtilisin
QQTVPWGITRVQAPAVHNRGITGSGVRVAILDSGISAHSDLNIRGGASFVPGEPTTADLNGHGTHVAGTVAALNNSIGVIGVAPNAELYAVKVLGANGRGSVSGIAQGLEWAATNNMHIANMSLGSDFPSSTLERAVNYATSRDVLVIAATGNNGSGSVGYPARYANAMAVGATDQNNRRANFSQYGTGIDIVAPGVNVQSTYPGNRYVSMNGTSMATPHVAGAAALVKQRYPSWNATQIRNHLKNTATNLGNSSQFGSGLVNAEAATR

SEQ ID NO: 206 - protein, 269 aa, artificial sequence
  B. gibsonii-clade subtilisin
QQTVPWGITRVQAPAVHNRGITGSGVRVAILDSGISAHSDLNIRGGASFVPGEPTTADLNGHGTHVAGTVAALNNSIGVIGVAPNAELYAVKVLGANGSGSVSGIAQGLEWAAANNMHIANMSLGSDFPSSTLERAVNYATSRDVLVIAATGNNGSGSVGYPARYANAMAVGATDQNNRRANFSQYGTGIDIVAPGVNVQSTYPGNRYVSMNGTSMATPHVAGAAALVKQRYPSWNATQIRNHLKNTATNLGNSSQFGSGLVNAEAATR

SEQ ID NO: 207 - protein, 269 aa, artificial sequence
  B. gibsonii-clade subtilisin
QQTVPWGITRVQAPAVHNRGITGSGVRVAILDSGISAHSDLNIRGGASFVPGEPTTADLNGHGTHVAGTVAALNNSIGVIGVAPNAELYAVKVLGANGSGSVSGIAQGLEWAATNNMHIANMSLGTDFPSSTLERAVNYATSRDVLVIAATGNNGSGSVGYPARYANAMAVGATDQNNRRANFSQYGTGIDIVAPGVNVQSTYPGNRYVSMNGTSMATPHVAGAAALVKQRYPSWNATQIRNHLKNTATNLGNSSQFGSGLVNAEAATR

SEQ ID NO: 208 - protein, 269 aa, artificial sequence
  B. gibsonii-clade subtilisin
QQTVPWGITRVQAPAVHNRGITGSGVRVAILDSGISAHSDLNIRGGASFVPGEPTTADLNGHGTHVAGTVAALNNSIGVIGVAPNAELYAVKVLGANGSGSVSGIAQGLEWAATNNMHIANMSLGSDAPSSTLERAVNYATSRDVLVIAATGNNGSGSVGYPARYANAMAVGATDQNNRRANFSQYGTGIDIVAPGVNVQSTYPGNRYVSMNGTSMATPHVAGAAALVKQRYPSWNATQIRNHLKNTATNLGNSSQFGSGLVNAEAATR

SEQ ID NO: 209 - protein, 269 aa, artificial sequence
  B. gibsonii-clade subtilisin
QQTVPWGITRVQAPAVHNRGITGSGVRVAILDSGISAHSDLNIRGGASFVPGEPTTADLNGHGTHVAGTVAALNNSIGVIGVAPNAELYAVKVLGANGSGSVSGIAQGLEWAATNNMHIANMSLGSDFPSSTLERAVNYATSRDVLVIAATGNNGSGSVGYPARYANAMAVGATDQNNRRANFSQYGTGIDIVAPGVNVQSTYPGNRYVSMNGTSMATPHVAGAAALVKQRYPSWNATQIRDHLKNTATNLGNSSQFGSGLVNAEAATR

SEQ ID NO: 210 - protein, 269 aa, artificial sequence
  B. gibsonii-clade subtilisin
QQTVPWGITRVQAPAVHNRGITGSGVRVAILDSGISAHSDLNIRGGASFVPGEPTTADLNGHGTHVAGTVAALNNSIGVIGVAPNAELYAVKVLGANGSGSVSGIAQGLEWAAQNNMHIANMSLGSDFPSSTLERAVNYATSRDVLVIAATGNNGSGSVGYPARYANAMAVGATDQNNRRANFSQYGTGIDIVAPGVNVQSTYPGNRYVSMNGTSMATPHVAGAAALVKQRYPSWNATQIRNHLKNTATNLGNSSQFGSGLVNAEAATR

SEQ ID NO: 211 - protein, 269 aa, artificial sequence
  B. gibsonii-clade subtilisin
QQTVPWGITRVQAPAVHNRGITGSGVRVAILDSGISAHSDLNIRGGASFVPGEPTTADLNGHGTHVAGTVAALNNSIGVIGVAPSAELYAVKVLGANGSGSVSGIAQGLEWAATNNMHIANMSLGSDFPSSTLERAVNYATSRDVLVIAATGNNGSGSVGYPARYANAMAVGATDQNNRRANFSQYGTGIDIVAPGVNVQSTYPGNRYVSMNGTSMATPHVAGAAALVKQRYPSWNATQIRNHLKNTATNLGNSSQFGSGLVNAEAATR

SEQ ID NO: 212 - protein, 269 aa, artificial sequence
  B. gibsonii-clade subtilisin
QQTVPWGITRVQAPAVHNRGITGSGVRVAILDSGISAHSDLNIRGGASFVPGEPTTADLNGHGTHVAGTVAALNNSIGVVGVAPNAELYAVKVLGANGSGSVSGIAQGLEWAATNNMHIANMSLGSDFPSSTLERAVNYATSRDVLVIAATGNNGSGSVGYPARYANAMAVGATDQNNRRANFSQYGTGIDIVAPGVNVQSTYPGNRYVSMNGTSMATPHVAGAAALVKQRYPSWNATQIRNHLKNTATNLGNSSQFGSGLVNAEAATR

SEQ ID NO: 213 - protein, 269 aa, artificial sequence
  B. gibsonii-clade subtilisin
QQTVPWGITRVQAPAVHNRGITGSGVRVAILDSGISAHEDLNIRGGASFVPGEPTTADLNGHGTHVAGTVAALNNSIGVIGVAPNADLYAVKVLGANGSGSVSGIAQGLEWAATNNMHIANMSLGSDFPSSTLERAVNYATSRDVLVIAATGNNGSGSVGYPARYANAMAVGATDQNNRRANFSQYGTGIDIVAPGVNVQSTYPGNRYVSMNGTSMATPHVAGAAALVKQRYPSWNATQIRNHLKNTATNLGNSSQFGSGLVNAEAATR

SEQ ID NO: 214 - protein, 269 aa, artificial sequence
  B. gibsonii-clade subtilisin
QQTVPWGITRVQAPAVHNRGITGSGVRVAILDSGISAHEDLNIRGGASFVPGEPTTADLNGHGTHVAGTVAALNNSIGVIGVAPNADLYAVKVLGANGSGSVSGIAQGLEWAATNNMHIANMSLGSDFPSSTLERAVNYATSRDVLVIAATGNNGSGSVGYPARYANAMAVGATDQNNRRANFSQYGTGIDIVAPGVNVQSTYPGNRYVSMNGTSMATPHVAGAAALVKQRYPSWNATQIRDHLKNTATNLGNSSQFGSGLVNAEAATR

SEQ ID NO: 215 - protein, 269 aa, artificial sequence
  B. gibsonii-clade subtilisin
QQTVPWGITRVQAPAVHNRGITGSGVRVAILDSGISAHEDLNIRGGASFVPGEPTTADLNGHGTHVAGTVAALNNSIGVIGVAPNADLYAVKVLGANGRGSVSGIAQGLEWAATNNMHIANMSLGSDAPSSTLERAVNYATSRDVLVIAATGNNGSGSVGYPARYANAMAVGATDQNNRRANFSQYGTGIDIVAPGVNVQSTYPGNRYVSMNGTSMATPHVAGAAALVKQRYPSWNATQIRNHLKNTATNLGNSSQFGSGLVNAEAATR

SEQ ID NO: 216 - protein, 269 aa, artificial sequence
  B. gibsonii-clade subtilisin
QQTVPWGITRVQAPAVHNRGITGSGVRVAILDSGISAHEDLNIRGGASFVPGEPTTADLNGHGTHVAGTVAALNNSIGVIGVAPNADLYAVKVLGANGRGSVSGIAQGLEWAATNNMHIANMSLGSDAPSSTLERAVNYATSRDVLVIAATGNNGSGSVGYPARYANAMAVGATDQNNRRANFSQYGTGIDIVAPGVNVQSTYPGNRYVSMNGTSMATPHVAGAAALVKQRYPSWNATQIRDHLKNTATNLGNSSQFGSGLVNAEAATR

SEQ ID NO: 217 - protein, 269 aa, artificial sequence
  B. gibsonii-clade subtilisin
QQTVPWGITRVQAPAVHNRGITGSGVRVAILDSGISAHSDLNIRGGASFVPGEPTYADLNGHGTHVAGTVAALNNSIGVIGVAPNAELYAVKVLGANGRGSVSGIAQGLEWAAQNNMHIANMSLGSDAPSSTLERAVNYATSRDVLVIAATGNNGSGSVGYPARYANAMAVGATDQNNRRANFSQYGTGIDIVAPGVNVQSTYPGNRYVSMNGTSMATPHVAGAAALVKQRYPSWNATQIRNHLKNTATNLGNSSQFGSGLVNAEAATR

SEQ ID NO: 218 - protein, 269 aa, artificial sequence
  B. gibsonii-clade subtilisin
QQTVPWGITRVQAPAVHNRGITGSGVRVAILDSGISAHEDLNIRGGASFVPGEPTTADLNGHGTHVAGTVAALNNSIGVIGVAPNADLYAVKVLGANGRGSVSGIAQGLEWAATNNMHIANMSLGTDFPSSTLERAVNYATSRDVLVIAATGNNGSGSVGYPARYANAMAVGATDQNNRRANFSQYGTGIDIVAPGVNVQSTYPGNRYVSMNGTSMATPHVAGAAALVKQRYPSWNATQIRNHLKNTATNLGNSSQFGSGLVNAEAATR

SEQ ID NO: 219 - protein, 269 aa, artificial sequence
  B. gibsonii-clade subtilisin
QQTVPWGITRVQAPAVHNRGITGSGVRVAILDSGISAHSDLNIRGGASFVPGEPTTADLNGHGTHVAGTVAALNNSIGVIGVAPNAELYAVKVLGANGRGSVSGIAQGLEWAATNNMHIANMSLGTDFPSSTLERAVNYATSRDVLVIAATGNNGSGSVGYPARYANAMAVGATDQNNRRANFSQYGTGIDIVAPGVNVQSTYPGNRYVSMNGTSMATPHVAGAAALVKQRYPSWNATQIRNHLKNTATNLGNSSQFGSGLVNAEAATR

SEQ ID NO: 220 - protein, 269 aa, artificial sequence
  B. gibsonii-clade subtilisin
QQTVPWGITRVQAPAVHNRGITGSGVRVAILDSGISAHSDLNIRGGASFVPGEPTTADLNGHGTHVAGTVAALNNSIGVIGVAPNAELYAVKVLGANGRGSVSGIAQGLEWAATNNMHIANMSLGTDFPSSTLERAVNYATSRDVLVIAATGNNGSGSVGYPARYANAMAVGATDQNNRRANFSQYGTGIDIVAPGVNVQSTYPGNRYVSMNGTSMATPHVAGAAALVKQRYPSWNATQIRDHLKNTATNLGNSSQFGSGLVNAEAATR

SEQ ID NO: 221 - protein, 269 aa, artificial sequence
  B. gibsonii-clade subtilisin
QQTVPWGITRVQAPAVHNRGITGSGVRVAILDSGISAHEDLNIRGGASFVPGEPTYADLNGHGTHVAGTVAALNNSIGVIGVAPNADLYAVKVLGANGSGSVSGIAQGLEWAAQNNMHIANMSLGSDFPSSTLERAVNYATSRDVLVIAATGNNGSGSVGYPARYANAMAVGATDQNNRRANFSQYGTGIDIVAPGVNVQSTYPGNRYVSMNGTSMATPHVAGAAALVKQRYPSWNATQIRNHLKNTATNLGNSSQFGSGLVNAEAATR

SEQ ID NO: 222 - protein, 269 aa, artificial sequence
  B. gibsonii-clade subtilisin
QQTVPWGITRVQAPAVHNRGITGSGVRVAILDSGISAHSDLNIRGGASFVPGEPTYADLNGHGTHVAGTVAALNNSIGVIGVAPNAELYAVKVLGANGSGSVSGIAQGLEWAAQNNMHIANMSLGSDFPSSTLERAVNYATSRDVLVIAATGNNGSGSVGYPARYANAMAVGATDQNNRRANFSQYGTGIDIVAPGVNVQSTYPGNRYVSMNGTSMATPHVAGAAALVKQRYPSWNATQIRDHLKNTATNLGNSSQFGSGLVNAEAATR

SEQ ID NO: 223 - protein, 269 aa, artificial sequence
  B. gibsonii-clade subtilisin
QQTVPWGITRVQAPAVHNRGITGSGVRVAILDSGISAHSDLNIRGGASFVPGEPTTADLNGHGTHVAGTVAALNNSIGVIGVAPNAELYAVKVLGANGRGSVSGIAQGLEWAATNNMHIANMSLGSDAPSSTLERAVNYATSRDVLVIAATGNNGSGSVGYPARYANAMAVGATDQNNRRANFSQYGTGIDIVAPGVNVQSTYPGNRYVSMNGTSMATPHVAGAAALVKQRYPSWNATQIRNHLKNTATNLGNSSQFGSGLVNAEAATR

SEQ ID NO: 224 - protein, 269 aa, artificial sequence
  B. gibsonii-clade subtilisin
QQTVPWGITRVQAPAVHNRGITGSGVRVAILDSGISAHSDLNIRGGASFVPGEPTYADLNGHGTHVAGTVAALNNSIGVIGVAPNAELYAVKVLGANGSGSVSGIAQGLEWAAQNNMHIANMSLGSDFPSSTLERAVNYATSRDVLVIAATGNNGSGSVGYPARYANAMAVGATDQNNRRANFSQYGTGIDIVAPGVNVQSTYPGNRYVSMNGTSMATPHVAGAAALVKQRYPSWNATQIRNHLKNTATNLGNSSQFGSGLVNAEAATR

SEQ ID NO: 225 - protein, 269 aa, artificial sequence
  B. gibsonii-clade subtilisin
QQTVPWGITRVQAPAVHNRGITGSGVRVAILDSGISAHSDLNIRGGASFVPGEPTYADLNGHGTHVAGTVAALNNSIGVIGVAPNAELYAVKVLGANGRGSVSGIAQGLEWAAQNNMHIANMSLGTDFPSSTLERAVNYATSRDVLVIAATGNNGSGSVGYPARYANAMAVGATDQNNRRANFSQYGTGIDIVAPGVNVQSTYPGNRYVSMNGTSMATPHVAGAAALVKQRYPSWNATQIRNHLKNTATNLGNSSQFGSGLVNAEAATR

SEQ ID NO: 226 - protein, 269 aa, artificial sequence
  B. gibsonii-clade subtilisin
QQTVPWGITRVQAPAVHNRGITGSGVRVAILDSGISAHSDLNIRGGASFVPGEPTTADLNGHGTHVAGTVAALNNSIGVIGVAPNAELYAVKVLGANGRGSVSGIAQGLEWAATNNMHIANMSLGSDAPSSTLERAVNYATSRDVLVIAATGNNGSGSVGYPARYANAMAVGATDQNNRRANFSQYGTGIDIVAPGVNVQSTYPGNRYVSMNGTSMATPHVAGAAALVKQRYPSWNATQIRDHLKNTATNLGNSSQFGSGLVNAEAATR

SEQ ID NO: 227 - protein, 269 aa, artificial sequence
  B. gibsonii-clade subtilisin
QQTVPWGITRVQAPAVHNRGITGSGVRVAILDSGISAHEDLNIRGGASFVPGEPTTADLNGHGTHVAGTVAALNNSIGVIGVAPNAELYAVKVLGANGRGSVSGIAQGLEWAATNNMHIANMSLGTDAPSSTLERAVNYATSRDVLVIAATGNNGSGSVGYPARYANAMAVGATDQNNRRANFSQYGTGIDIVAPGVNVQSTYPGNRYVSMNGTSMATPHVAGAAALVKQRYPSWNATQIRNHLKNTATNLGNSSQFGSGLVNAEAATR

SEQ ID NO: 228 - protein, 269 aa, artificial sequence
  B. gibsonii-clade subtilisin
QQTVPWGITRVQAPAVHNRGITGSGVRVAILDSGISAHEDLNIRGGASFVPGEPTYADLNGHGTHVAGTVAALNNSIGVIGVAPNAELYAVKVLGANGRGSVSGIAQGLEWAATNNMHIANMSLGTDAPSSTLERAVNYATSRDVLVIAATGNNGSGSVGYPARYANAMAVGATDQNNRRANFSQYGTGIDIVAPGVNVQSTYPGNRYVSMNGTSMATPHVAGAAALVKQRYPSWNATQIRNHLKNTATNLGNSSQFGSGLVNAEAATR

SEQ ID NO: 229 - protein, 269 aa, artificial sequence
  B. gibsonii-clade subtilisin
QQTVPWGITRVQAPAVHNRGITGSGVRVAILDSGISAHSDLNIRGGASFVPGEPTTADLNGHGTHVAGTVAALNNSIGVIGVAPNAELYAVKVLGANGSGSVSGIAQGLEWAATNNMHIANMSLGTDAPSSTLERAVNYATSRDVLVIAATGNNGSGSVGYPARYANAMAVGATDQNNRRANFSQYGTGIDIVAPGVNVQSTYPGNRYVSMNGTSMATPHVAGAAALVKQRYPSWNATQIRNHLKNTATNLGNSSQFGSGLVNAEAATR

SEQ ID NO: 230 - protein, 269 aa, artificial sequence
  B. gibsonii-clade subtilisin
QQTVPWGITRVQAPAVHNRGITGSGVRVAILDSGISAHEDLNIRGGASFVPGEPTTADLNGHGTHVAGTVAALNNSIGVIGVAPNAELYAVKVLGANGRGSVSGIAQGLEWAATNNMHIANMSLGTDFPSSTLERAVNYATSRDVLVIAATGNNGSGSVGYPARYANAMAVGATDQNNRRANFSQYGTGIDIVAPGVNVQSTYPGNRYVSMNGTSMATPHVAGAAALVKQRYPSWNATQIRNHLKNTATNLGNSSQFGSGLVNAEAATR

SEQ ID NO: 231 - protein, 269 aa, artificial sequence
  B. gibsonii-clade subtilisin
QQTVPWGITRVQAPAVHNRGITGSGVRVAILDSGISAHEDLNIRGGASFVPGEPTTADLNGHGTHVAGTVAALNNSIGVIGVAPNAELYAVKVLGANGRGSVSGIAQGLEWAATNNMHIANMSLGSDAPSSTLERAVNYATSRDVLVIAATGNNGSGSVGYPARYANAMAVGATDQNNRRANFSQYGTGIDIVAPGVNVQSTYPGNRYVSMNGTSMATPHVAGAAALVKQRYPSWNATQIRNHLKNTATNLGNSSQFGSGLVNAEAATR

SEQ ID NO: 232 - protein, 269 aa, artificial sequence
  B. gibsonii-clade subtilisin
QQTVPWGITRVQAPAVHNRGITGSGVRVAILDSGISAHSDLNIRGGASFVPGEPTTADLNGHGTHVAGTVAALNNSIGVIGVAPNAELYAVKVLGANGRGSVSGIAQGLEWAATNNMHIANMSLGTDAPSSTLERAVNYATSRDVLVIAATGNNGSGSVGYPARYANAMAVGATDQNNRRANFSQYGTGIDIVAPGVNVQSTYPGNRYVSMNGTSMATPHVAGAAALVKQRYPSWNATQIRNHLKNTATNLGNSSQFGSGLVNAEAATR

SEQ ID NO: 233 - protein, 269 aa, artificial sequence
  B. gibsonii-clade subtilisin
QQTVPWGITRVQAPAVHNRGITGSGVRVAILDSGISAHEDLNIRGGVSFVPGEPTYADLNGHGTHVAGTVAALNNSIGVIGVAPNADLYAVKVLGANGRGSVSGIAQGLEWAAQNNMHIANMSLGTDAPSSTLERAVNYATSRDVLVIAATGNNGSGSVGYPARYANAMAVGATDQNNRRANFSQYGTGIDIVAPGVNVQSTYPGNRYVSMNGTSMATPHVAGAAALVKQRYPSWNATQIRDHLKNTATNLGNSSQFGSGLVNAEAATR

SEQ ID NO: 234 - protein, 269 aa, artificial sequence
  B. gibsonii-clade subtilisin
QQTVPWGITRVQAPAVHNRGITGSGVRVAILDSGISTHEDLNIRGGASFVPGEPTTADLNGHGTHVAGTVAALNNSIGVIGVAPNAELYAVKVLGANGRGSVSGIAQGLEWAAQNNMHIANMSLGTDAPSSTLERAVNYATSRDVLVIAATGNNGSGSVGYPARYANAMAVGATDQNNRRANFSQYGTGIDIVAPGVNVQSTYPGNRYVSMNGTSMATPHVAGAAALVKQRYPSWNATQIRDHLKNTATNLGNSSQFGSGLVNAEAATR

SEQ ID NO: 235 - protein, 269 aa, artificial sequence
  B. gibsonii-clade subtilisin
QQTVPWGITRVQAPAVHNRGITGSGVRVAILDSGISAHEDLNIRGGASFVPGEPTTADLNGHGTHVAGTVAALNNSIGVIGVAPNADLYAVKVLGANGRGSVSGIAQGLEWAATNNMHIANMSLGTDAPSSTLERAVNYATSRDVLVIAATGNNGSGSVGYPARYANAMAVGATDQNNRRANFSQYGTGIDIVAPGVNVQSTYPGNRYVSMNGTSMATPHVAGAAALVKQRYPSWNATQIRNHLKNTATNLGNSSQFGSGLVNAEAATR

SEQ ID NO: 236 - protein, 269 aa, artificial sequence
  B. gibsonii-clade subtilisin
QQTVPWGITRVQAPAVHNRGITGSGVRVAILDSGISAHEDLNIRGGASFVPGEPTYADLNGHGTHVAGTVAALNNSIGVIGVAPNADLYAVKVLGANGRGSVSGIAQGLEWAATNNMHIANMSLGTDAPSSTLERAVNYATSRDVLVIAATGNNGSGSVGYPARYANAMAVGATDQNNRRANFSQYGTGIDIVAPGVNVQSTYPGNRYVSMNGTSMATPHVAGAAALVKQRYPSWNATQIRNHLKNTATNLGNSSQFGSGLVNAEAATR

SEQ ID NO: 237 - protein, 269 aa, artificial sequence
  B. gibsonii-clade subtilisin
QQTVPWGITRVQAPAVHNRGITGSGVRVAILDSGISTHEDLNIRGGASFVPGEPTTADLNGHGTHVAGTVAALNNSIGVVGVAPSADLYAVKVLGANGRGSVSGIAQGLEWAAQNNMHIANMSLGTDAPSSTLERAVNYATSRDVLVIAATGNNGSGSVGYPARYANAMAVGATDQNNRRANFSQYGTGIDIVAPGVNVQSTYPGNRYVSMNGTSMATPHVAGAAALVKQRYPSWNATQIRDHLKNTATNLGNSSQFGSGLVNAEAATR

SEQ ID NO: 238 - protein, 269 aa, artificial sequence
  B. gibsonii-clade subtilisin
QQTVPWGITRVQAPAVHNRGITGSGVRVAILDSGISTHEDLNIRGGASFVPGEPTYADLNGHGTHVAGTVAALNNSIGVIGVAPNAELYAVKVLGANGRGSVSGIAQGLEWAATNNMHIANMSLGTDAPSSTLERAVNYATSRDVLVIAATGNNGSGSVGYPARYANAMAVGATDQNNRRANFSQYGTGIDIVAPGVNVQSTYPGNRYVSMNGTSMATPHVAGAAALVKQRYPSWNATQIRDHLKNTATNLGNSSQFGSGLVNAEAATR

SEQ ID NO: 239 - protein, 269 aa, artificial sequence
  B. gibsonii-clade subtilisin
QQTVPWGITRVQAPAVHNRGITGSGVRVAILDSGISTHEDLNIRGGVSFVPGEPTTADLNGHGTHVAGTVAALNNSIGVVGVAPSADLYAVKVLGANGRGSVSGIAQGLEWAAANNMHIANMSLGTDAPSSTLERAVNYATSRDVLVIAATGNNGSGSVGYPARYANAMAVGATDQNNRRANFSQYGTGIDIVAPGVNVQSTYPGNRYVSMNGTSMATPHVAGAAALVKQRYPSWNATQIRNHLKNTATNLGNSSQFGSGLVNAEAATR

SEQ ID NO: 240 - protein, 269 aa, artificial sequence
  B. gibsonii-clade subtilisin
QQTVPWGITRVQAPAVHNRGITGSGVRVAILDSGISTHEDLNIRGGASFVPGEPTTADLNGHGTHVAGTVAALNNSIGVIGVAPNADLYAVKVLGANGRGSVSGIAQGLEWAAANNMHIANMSLGSDAPSSTLERAVNYATSRDVLVIAATGNNGSGSVGYPARYANAMAVGATDQNNRRANFSQYGTGIDIVAPGVNVQSTYPGNRYVSMNGTSMATPHVAGAAALVKQRYPSWNATQIRNHLKNTATNLGNSSQFGSGLVNAEAATR

SEQ ID NO: 241 - protein, 269 aa, artificial sequence
  B. gibsonii-clade subtilisin
QQTVPWGITRVQAPAVHNRGITGSGVRVAILDSGISTHEDLNIRGGVSFVPGEPTYADLNGHGTHVAGTVAALNNSIGVIGVAPNAELYAVKVLGANGRGSVSGIAQGLEWAAQNNMHIANMSLGTDAPSSTLERAVNYATSRDVLVIAATGNNGSGSVGYPARYANAMAVGATDQNNRRANFSQYGTGIDIVAPGVNVQSTYPGNRYVSMNGTSMATPHVAGAAALVKQRYPSWNATQIRNHLKNTATNLGNSSQFGSGLVNAEAATR

SEQ ID NO: 242 - protein, 269 aa, artificial sequence
  B. gibsonii-clade subtilisin
QQTVPWGITRVQAPAVHNRGITGSGVRVAILDSGISAHEDLNIRGGVSFVPGEPTTADLNGHGTHVAGTVAALNNSIGVIGVAPNADLYAVKVLGANGRGSVSGIAQGLEWAAQNNMHIANMSLGTDAPSSTLERAVNYATSRDVLVIAATGNNGSGSVGYPARYANAMAVGATDQNNRRANFSQYGTGIDIVAPGVNVQSTYPGNRYVSMNGTSMATPHVAGAAALVKQRYPSWNATQIRDHLKNTATNLGNSSQFGSGLVNAEAATR

SEQ ID NO: 243 - protein, 269 aa, artificial sequence
  B. gibsonii-clade subtilisin
QQTVPWGITRVQAPAVHNRGITGSGVRVAILDSGISAHEDLNIRGGASFVPGEPTTADLNGHGTHVAGTVAALNNSIGVIGVAPSAELYAVKVLGANGRGSVSGIAQGLEWAATNNMHIANMSLGSDAPSSTLERAVNYATSRDVLVIAATGNNGSGSVGYPARYANAMAVGATDQNNRRANFSQYGTGIDIVAPGVNVQSTYPGNRYVSMNGTSMATPHVAGAAALVKQRYPSWNATQIRNHLKNTATNLGNSSQFGSGLVNAEAATR

SEQ ID NO: 244 - protein, 269 aa, artificial sequence
  B. gibsonii-clade subtilisin
QQTVPWGITRVQAPAVHNRGITGSGVRVAILDSGISAHEDLNIRGGASFVPGEPTTADLNGHGTHVAGTVAALNNSIGVIGVAPNAELYAVKVLGANGRGSVSGIAQGLEWAAQNNMHIANMSLGSDAPSSTLERAVNYATSRDVLVIAATGNNGSGSVGYPARYANAMAVGATDQNNRRANFSQYGTGIDIVAPGVNVQSTYPGNRYVSMNGTSMATPHVAGAAALVKQRYPSWNATQIRNHLKNTATNLGNSSQFGSGLVNAEAATR

SEQ ID NO: 245 - protein, 269 aa, artificial sequence
  B. gibsonii-clade subtilisin
QQTVPWGITRVQAPAVHNRGITGSGVRVAILDSGISTHEDLNIRGGASFVPGEPTYADLNGHGTHVAGTVAALNNSIGVIGVAPNAELYAVKVLGANGRGSVSGIAQGLEWAAQNNMHIANMSLGTDAPSSTLERAVNYATSRDVLVIAATGNNGSGSVGYPARYANAMAVGATDQNNRRANFSQYGTGIDIVAPGVNVQSTYPGNRYVSMNGTSMATPHVAGAAALVKQRYPSWNATQIRDHLKNTATNLGNSSQFGSGLVNAEAATR

SEQ ID NO: 246 - protein, 269 aa, artificial sequence
  B. gibsonii-clade subtilisin
QQTVPWGITRVQAPAVHNRGITGSGVRVAILDSGISTHEDLNIRGGVSFVPGEPTYADLNGHGTHVAGTVAALNNSIGVIGVAPNAELYAVKVLGANGRGSVSGIAQGLEWAAANNMHIANMSLGTDAPSSTLERAVNYATSRDVLVIAATGNNGSGSVGYPARYANAMAVGATDQNNRRANFSQYGTGIDIVAPGVNVQSTYPGNRYVSMNGTSMATPHVAGAAALVKQRYPSWNATQIRNHLKNTATNLGNSSQFGSGLVNAEAATR

SEQ ID NO: 247 - protein, 269 aa, artificial sequence
  B. gibsonii-clade subtilisin
QQTVPWGITRVQAPAVHNRGITGSGVRVAILDSGISAHEDLNIRGGVSFVPGEPTYADLNGHGTHVAGTVAALNNSIGVIGVAPNADLYAVKVLGANGRGSVSGIAQGLEWAAANNMHIANMSLGTDAPSSTLERAVNYATSRDVLVIAATGNNGSGSVGYPARYANAMAVGATDQNNRRANFSQYGTGIDIVAPGVNVQSTYPGNRYVSMNGTSMATPHVAGAAALVKQRYPSWNATQIRDHLKNTATNLGNSSQFGSGLVNAEAATR

SEQ ID NO: 248 - protein, 269 aa, artificial sequence
  B. gibsonii-clade subtilisin
QQTVPWGITRVQAPAVHNRGITGSGVRVAILDSGISTHEDLNIRGGASFVPGEPTYADLNGHGTHVAGTVAALNNSIGVIGVAPSAELYAVKVLGANGRGSVSGIAQGLEWAAQNNMHIANMSLGTDAPSSTLERAVNYATSRDVLVIAATGNNGSGSVGYPARYANAMAVGATDQNNRRANFSQYGTGIDIVAPGVNVQSTYPGNRYVSMNGTSMATPHVAGAAALVKQRYPSWNATQIRDHLKNTATNLGNSSQFGSGLVNAEAATR

SEQ ID NO: 249 - protein, 269 aa, artificial sequence
  B. gibsonii-clade subtilisin
QQTVPWGITRVQAPAVHNRGITGSGVRVAILDSGISTHEDLNIRGGVSFVPGEPTYADLNGHGTHVAGTVAALNNSIGVIGVAPNADLYAVKVLGANGRGSVSGIAQGLEWAAANNMHIANMSLGTDAPSSTLERAVNYATSRDVLVIAATGNNGSGSVGYPARYANAMAVGATDQNNRRANFSQYGTGIDIVAPGVNVQSTYPGNRYVSMNGTSMATPHVAGAAALVKQRYPSWNATQIRDHLKNTATNLGNSSQFGSGLVNAEAATR

SEQ ID NO: 250 - protein, 269 aa, artificial sequence
  B. gibsonii-clade subtilisin
QQTVPWGITRVQAPAVHNRGITGSGVRVAILDSGISAHEDLNIRGGVSFVPGEPTYADLNGHGTHVAGTVAALNNSIGVIGVAPSADLYAVKVLGANGRGSVSGIAQGLEWAAQNNMHIANMSLGTDAPSSTLERAVNYATSRDVLVIAATGNNGSGSVGYPARYANAMAVGATDQNNRRANFSQYGTGIDIVAPGVNVQSTYPGNRYVSMNGTSMATPHVAGAAALVKQRYPSWNATQIRNHLKNTATNLGNSSQFGSGLVNAEAATR

SEQ ID NO: 251 - protein, 269 aa, artificial sequence
  B. gibsonii-clade subtilisin
QQTVPWGITRVQAPAVHNRGITGSGVRVAILDSGISTHEDLNIRGGASFVPGEPTYADLNGHGTHVAGTVAALNNSIGVIGVAPSADLYAVKVLGANGRGSVSGIAQGLEWAAQNNMHIANMSLGSDAPSSTLERAVNYATSRDVLVIAATGNNGSGSVGYPARYANAMAVGATDQNNRRANFSQYGTGIDIVAPGVNVQSTYPGNRYVSMNGTSMATPHVAGAAALVKQRYPSWNATQIRNHLKNTATNLGNSSQFGSGLVNAEAATR

SEQ ID NO: 252 - protein, 269 aa, artificial sequence
  B. gibsonii-clade subtilisin
QQTVPWGITRVQAPAVHNRGITGSGVRVAILDSGISAHEDLNIRGGASFVPGEPTYADLNGHGTHVAGTVAALNNSIGVIGVAPNAELYAVKVLGANGRGSVSGIAQGLEWAATNNMHIANMSLGSDAPSSTLERAVNYATSRDVLVIAATGNNGSGSVGYPARYANAMAVGATDQNNRRANFSQYGTGIDIVAPGVNVQSTYPGNRYVSMNGTSMATPHVAGAAALVKQRYPSWNATQIRNHLKNTATNLGNSSQFGSGLVNAEAATR

SEQ ID NO: 253 - protein, 269 aa, artificial sequence
  B. gibsonii-clade subtilisin
QQTVPWGITRVQAPAVHNRGITGSGVRVAILDSGISAHEDLNIRGGVSFVPGEPTTADLNGHGTHVAGTVAALNNSIGVVGVAPNADLYAVKVLGANGRGSVSGIAQGLEWAAANNMHIANMSLGTDAPSSTLERAVNYATSRDVLVIAATGNNGSGSVGYPARYANAMAVGATDQNNRRANFSQYGTGIDIVAPGVNVQSTYPGNRYVSMNGTSMATPHVAGAAALVKQRYPSWNATQIRDHLKNTATNLGNSSQFGSGLVNAEAATR

SEQ ID NO: 254 - protein, 269 aa, artificial sequence
  B. gibsonii-clade subtilisin
QQTVPWGITRVQAPAVHNRGITGSGVRVAILDSGISTHEDLNIRGGASFVPGEPTYADLNGHGTHVAGTVAALNNSIGVIGVAPSADLYAVKVLGANGRGSVSGIAQGLEWAAANNMHIANMSLGTDAPSSTLERAVNYATSRDVLVIAATGNNGSGSVGYPARYANAMAVGATDQNNRRANFSQYGTGIDIVAPGVNVQSTYPGNRYVSMNGTSMATPHVAGAAALVKQRYPSWNATQIRDHLKNTATNLGNSSQFGSGLVNAEAATR

SEQ ID NO: 255 - protein, 269 aa, artificial sequence
  B. gibsonii-clade subtilisin
QQTVPWGITRVQAPAVHNRGITGSGVRVAILDSGISAHEDLNIRGGASFVPGEPTTADLNGHGTHVAGTVAALNNSIGVIGVAPNAELYAVKVLGANGRGSVSGIAQGLEWAAANNMHIANMSLGTDFPSSTLERAVNYATSRDVLVIAATGNNGSGSVGYPARYANAMAVGATDQNNRRANFSQYGTGIDIVAPGVNVQSTYPGNRYVSMNGTSMATPHVAGAAALVKQRYPSWNATQIRNHLKNTATNLGNSSQFGSGLVNAEAATR

SEQ ID NO: 256 - protein, 269 aa, artificial sequence
  B. gibsonii-clade subtilisin
QQTVPWGITRVQAPAVHNRGITGSGVRVAILDSGISAHEDLNIRGGASFVPGEPTTADLNGHGTHVAGTVAALNNSIGVIGVAPNAELYAVKVLGANGRGSVSGIAQGLEWAAQNNMHIANMSLGTDAPSSTLERAVNYATSRDVLVIAATGNNGSGSVGYPARYANAMAVGATDQNNRRANFSQYGTGIDIVAPGVNVQSTYPGNRYVSMNGTSMATPHVAGAAALVKQRYPSWNATQIRDHLKNTATNLGNSSQFGSGLVNAEAATR

SEQ ID NO: 257 - protein, 269 aa, artificial sequence
  Consensus sequence Figure 14
  MISC_FEATURE (114)..(114): Xaa can be any amino acid
QQTVPWGITRVQAPAVHNRGITGSGVRVAILDSGISAHEDLNIRGGASFVPGEPTTADLNGHGTHVAGTVAALNNSIGVIGVAPNAELYAVKVLGANGRGSVSGIAQGLEWAAXNNMHIANMSLGTDAPSSTLERAVNYATSRDVLVIAATGNNGSGSVGYPARYANAMAVGATDQNNRRANFSQYGTGIDIVAPGVNVQSTYPGNRYVSMNGTSMATPHVAGAAALVKQRYPSWNATQIRNHLKNTATNLGNSSQFGSGLVNAEAATR